European Patent Specification EP 3 910 073 B1, published March 6, 2024. Title: SPLICE VARIANTS ASSOCIATED WITH NEOMORPHIC SF3B1 MUTANTS. Applicant: EISAI R&D MANAGEMENT CO., LTD. YU, LIHUA LIM, KIAN HUAT FEALA, JACOB D. BUONAMICI, SILVIA MIZUI, YOSHIHARU SMITH, PETER G. ZHU, PING PARK, EUNICE SUN SEILER, MICHAEL W. FEKKES, MARCO PETER. The sequence listing filed with the application follows.

SEQUENCE LISTING (1200 sequences)

SEQ ID NO: 1 - DNA, 40 bp, Homo sapiens
agcaagtagaagtctataaaatttacccccagatacagct

SEQ ID NO: 2 - DNA, 40 bp, Homo sapiens
agcaagtagaagtctataaaatacagctggctgaaataac

SEQ ID NO: 3 - DNA, 40 bp, Homo sapiens
cgggccgcatcatccgggagagcactgtgttccagctgcc

SEQ ID NO: 4 - DNA, 40 bp, Homo sapiens
cgggccgcatcatccgggagctgcccggtgtccaccctga

SEQ ID NO: 5 - DNA, 40 bp, Homo sapiens
ctggagccggcgggaaggagtgtgctggttcctctcccca

SEQ ID NO: 6 - DNA, 40 bp, Homo sapiens
ctggagccggcgggaaggaggcaagctgcagcagttcgag

SEQ ID NO: 7 - DNA, 40 bp, Homo sapiens
ggcccttttgtcctcactagcatttctgttctgacaggtt

SEQ ID NO: 8 - DNA, 40 bp, Homo sapiens
ggcccttttgtcctcactaggttcttggcatggagctgag

SEQ ID NO: 9 - DNA, 40 bp, Homo sapiens
tgggaggagcatgtcaacagagtttcccttataggactgg

SEQ ID NO: 10 - DNA, 40 bp, Homo sapiens
tgggaggagcatgtcaacaggactggctggacaatggccc

SEQ ID NO: 11 - DNA, 40 bp, Homo sapiens
gatggtggatgaacccacagtttttttttttcaggtatat

SEQ ID NO: 12 - DNA, 40 bp, Homo sapiens
gatggtggatgaacccacaggtatatgtcctcattttcct

SEQ ID NO: 13 - DNA, 40 bp, Homo sapiens
tacctctggttcctgtgcagtcttcgcccctcttttctta

SEQ ID NO: 14 - DNA, 40 bp, Homo sapiens
tacctctggttcctgtgcagttctgtggcacttgccctgg

SEQ ID NO: 15 - DNA, 40 bp, Homo sapiens
ttggaccggaaaagactttgagtctctttttgcagatgat

SEQ ID NO: 16 - DNA, 40 bp, Homo sapiens
ttggaccggaaaagactttgatgatggatgccaaccagcg

SEQ ID NO: 17 - DNA, 40 bp, Homo sapiens
acccaagccttgaggtttcatttccccctcccaggatttc

SEQ ID NO: 18 - DNA, 40 bp, Homo sapiens
acccaagccttgaggtttcagcctgggcagcatggccgta

SEQ ID NO: 19 - DNA, 40 bp, Homo sapiens
agcattgctagaagcagcagcttttgcagatcctgaggta

SEQ ID NO: 20 - DNA, 40 bp, Homo sapiens
agcattgctagaagcagcaggaattggcaaattgtcaact

SEQ ID NO: 21 - DNA, 40 bp, Homo sapiens
caagtatatgactgaagaagatcctgaattccagcaaaac

SEQ ID NO: 22 - DNA, 40 bp, Homo sapiens
caagtatatgactgaagaaggtgagcctttttctcaagag

SEQ ID NO: 23 - DNA, 40 bp, Homo sapiens
tgcagtttggtcagtctgtgccttcctcacccctctcctc

SEQ ID NO: 24 - DNA, 40 bp, Homo sapiens
tgcagtttggtcagtctgtgggctctgtggtatatgactg

SEQ ID NO: 25 - DNA, 40 bp, Homo sapiens
tctttggaaaatctaatcaattttctgcctataggggaag

SEQ ID NO: 26 - DNA, 40 bp, Homo sapiens
tctttggaaaatctaatcaagggaaggaagatctatgaac

SEQ ID NO: 27 - DNA, 40 bp, Homo sapiens
gtatcaaagtgtggactgagatttgtcttcctttaggatt

SEQ ID NO: 28 - DNA, 40 bp, Homo sapiens
gtatcaaagtgtggactgaggattccattgcaaagccaca

SEQ ID NO: 29 - DNA, 40 bp, Homo sapiens
agaactgcacctacacacagccctgttcacaggtgcagac

SEQ ID NO: 30 - DNA, 40 bp, Homo sapiens
agaactgcacctacacacaggtgcagacccgcagctctga

SEQ ID NO: 31 - DNA, 40 bp, Homo sapiens
ggagcagtgcagttgtgaaatcattacttctagatgatgc

SEQ ID NO: 32 - DNA, 40 bp, Homo sapiens
ggagcagtgcagttgtgaaagttttgattcatggattcac

SEQ ID NO: 33 - DNA, 40 bp, Homo sapiens
ctatttcactctcccccgaacctatccaggttcctcctcc

SEQ ID NO: 34 - DNA, 40 bp, Homo sapiens
ctatttcactctcccccgaaatgagcccatccagccaatt

SEQ ID NO: 35 - DNA, 40 bp, Homo sapiens
tttgcagggaatgggctacatccccttggttctctgttac

SEQ ID NO: 36 - DNA, 40 bp, Homo sapiens
tttgcagggaatgggctacataccatctgccagcatgact

SEQ ID NO: 37 - DNA, 40 bp, Homo sapiens
tgaccacggagtacctggggcccttttttctctttccttc

SEQ ID NO: 38 - DNA, 40 bp, Homo sapiens
tgaccacggagtacctggggatcatgaccaacacggggaa

SEQ ID NO: 39 - DNA, 40 bp, Homo sapiens
agacctaccagaaggctatgtgtttattaattttacagaa

SEQ ID NO: 40 - DNA, 40 bp, Homo sapiens
agacctaccagaaggctatgaacagaggacaacgcaacaa

SEQ ID NO: 41 - DNA, 40 bp, Homo sapiens
atttggactcgctagcaatgatgtctgtttatttttagag

SEQ ID NO: 42 - DNA, 40 bp, Homo sapiens
atttggactcgctagcaatgagcatgacctctcaatggca

SEQ ID NO: 43 - DNA, 40 bp, Homo sapiens
catgtggaatcccaatgccggcccctgtcctcctccccca

SEQ ID NO: 44 - DNA, 40 bp, Homo sapiens
catgtggaatcccaatgccgggcagccagggccaaatcca

SEQ ID NO: 45 - DNA, 40 bp, Homo sapiens
ctgggaggtggcattcaaagccccaccttttgtctcccca

SEQ ID NO: 46 - DNA, 40 bp, Homo sapiens
ctgggaggtggcattcaaaggctcttcagaggtgttcctg

SEQ ID NO: 47 - DNA, 40 bp, Homo sapiens
ggatgaccgggatgcctcagtcactttacagctgcatcgt

SEQ ID NO: 48 - DNA, 40 bp, Homo sapiens
ggatgaccgggatgcctcagatggggaggatgagaagccc

SEQ ID NO: 49 - DNA, 40 bp, Homo sapiens
acatgaaggtggacggagaggctcccctcccaccccaggt

SEQ ID NO: 50 - DNA, 40 bp, Homo sapiens
acatgaaggtggacggagaggtactgaggacaaatcagtt

SEQ ID NO: 51 - DNA, 40 bp, Homo sapiens
agagaagtcgtttcattcaagtcagctaagacacaagcag

SEQ ID NO: 52 - DNA, 40 bp, Homo sapiens
agagaagtcgtttcattcaagttggtgtaatcagctgggg

SEQ ID NO: 53 - DNA, 40 bp, Homo sapiens
tcactcaaacagtaaacgagttttatcatttacaggtatg

SEQ ID NO: 54 - DNA, 40 bp, Homo sapiens
tcactcaaacagtaaacgaggtatgtgacgcattcccaga

SEQ ID NO: 55 - DNA, 40 bp, Homo sapiens
cgatctcccaaaaggagaagtctgaccagtcttttctaca

SEQ ID NO: 56 - DNA, 40 bp, Homo sapiens
cgatctcccaaaaggagaagcccctcccctcgccgagaaa

SEQ ID NO: 57 - DNA, 40 bp, Homo sapiens
ttattttacacaatccaaagccagttgcagggtctgatga

SEQ ID NO: 58 - DNA, 40 bp, Homo sapiens
ttattttacacaatccaaagcttatggtgcattaccagcc

SEQ ID NO: 59 - DNA, 40 bp, Homo sapiens
tgcctgtggacatcaccaagcctcgtcctccccaggtgcc

SEQ ID NO: 60 - DNA, 40 bp, Homo sapiens
tgcctgtggacatcaccaaggtgccgcctgcccctgtcaa

SEQ ID NO: 61 - DNA, 40 bp, Homo sapiens
agttagaatccaaaccagagtgttgtcttttctcccccca

SEQ ID NO: 62 - DNA, 40 bp, Homo sapiens
agttagaatccaaaccagagctcctggtacagtttgttca

SEQ ID NO: 63 - DNA, 40 bp, Homo sapiens
atatgctggaatggttccttgtcacaatgcacgacacccg

SEQ ID NO: 64 - DNA, 40 bp, Homo sapiens
atatgctggaatggttccttaccgaccgctcgggagctcg

SEQ ID NO: 65 - DNA, 40 bp, Homo sapiens
atcagaaattcgtacaacaggtttcttttaaagctcctgg

SEQ ID NO: 66 - DNA, 40 bp, Homo sapiens
atcagaaattcgtacaacagctcctggagctttttgatag

SEQ ID NO: 67 - DNA, 40 bp, Homo sapiens
aaatgaagaaactcctaaagcctctctctttctttgttta

SEQ ID NO: 68 - DNA, 40 bp, Homo sapiens
aaatgaagaaactcctaaagataaagtcctgtttatgacc

SEQ ID NO: 69 - DNA, 40 bp, Homo sapiens
cataaaattctaacagctaattctctttcctctgtcttca

SEQ ID NO: 70 - DNA, 40 bp, Homo sapiens
cataaaattctaacagctaagcaagcactgagcgaggtga

SEQ ID NO: 71 - DNA, 40 bp, Homo sapiens
gcctgcctttgatgccctggattttgcccgaacaggtcag

SEQ ID NO: 72 - DNA, 40 bp, Homo sapiens
gcctgcctttgatgccctgggtcagttgactggcggctat

SEQ ID NO: 73 - DNA, 40 bp, Homo sapiens
ccaagctggtgtgcgcacaggcctctcttcccgcccaggc

SEQ ID NO: 74 - DNA, 40 bp, Homo sapiens
ccaagctggtgtgcgcacaggcatcatcgggaagaagcac

SEQ ID NO: 75 - DNA, 40 bp, Homo sapiens
ctcctttgggtttgggccaggccccaggtcccaccacagc

SEQ ID NO: 76 - DNA, 40 bp, Homo sapiens
ctcctttgggtttgggccagtgacctggcttgtcctcagc

SEQ ID NO: 77 - DNA, 40 bp, Homo sapiens
aatattgctttaccaaacagggaccccttccccttcccca

SEQ ID NO: 78 - DNA, 40 bp, Homo sapiens
aatattgctttaccaaacaggtcacggaggagtaaagtat

SEQ ID NO: 79 - DNA, 40 bp, Homo sapiens
cagttataaactctagagtgagtttattttccttttacaa

SEQ ID NO: 80 - DNA, 40 bp, Homo sapiens
cagttataaactctagagtgcttactgcagtgcatggtat

SEQ ID NO: 81 - DNA, 40 bp, Homo sapiens
gcctgccccggaaactcaagatgttcagcgatgcaggtag

SEQ ID NO: 82 - DNA, 40 bp, Homo sapiens
gcctgccccggaaactcaagatggcggtgggaccccccga

SEQ ID NO: 83 - DNA, 40 bp, Homo sapiens
ttcaggaggtggagcaccagataatttttttcctcacaca

SEQ ID NO: 84 - DNA, 40 bp, Homo sapiens
ttcaggaggtggagcaccagttgcggtcttgtagtaagag

SEQ ID NO: 85 - DNA, 40 bp, Homo sapiens
ggatccttcacccgtgtctgtctttgcagacaggttctgt

SEQ ID NO: 86 - DNA, 40 bp, Homo sapiens
ggatccttcacccgtgtctggacccgtgcatctcttccga

SEQ ID NO: 87 - DNA, 40 bp, Homo sapiens
atttggatcctgtgttcctctttttttctgttaaagatac

SEQ ID NO: 88 - DNA, 40 bp, Homo sapiens
atttggatcctgtgttcctcatacaactagaccaaaacga

SEQ ID NO: 89 - DNA, 40 bp, Homo sapiens
agatgtcaggtgggagaaagcctttgattgtcttttcagc

SEQ ID NO: 90 - DNA, 40 bp, Homo sapiens
agatgtcaggtgggagaaagctgttggagacacagttgca

SEQ ID NO: 91 - DNA, 40 bp, Homo sapiens
agaaagagcataaattggaaatattggacatgggcgtatc

SEQ ID NO: 92 - DNA, 40 bp, Homo sapiens
agaaagagcataaattggaagagtacaagcgcaagctagc

SEQ ID NO: 93 - DNA, 40 bp, Homo sapiens
tcagccctctgaactacaaaggtgtttgttcacagagatc

SEQ ID NO: 94 - DNA, 40 bp, Homo sapiens
tcagccctctgaactacaaaacagaagagcctgcaagtga

SEQ ID NO: 95 - DNA, 40 bp, Homo sapiens
ccggggccttcgtgagaccgcttgttttctgcaggtgcag

SEQ ID NO: 96 - DNA, 40 bp, Homo sapiens
ccggggccttcgtgagaccggtgcaggcctggggtagtct

SEQ ID NO: 97 - DNA, 40 bp, Homo sapiens
caagtccatctctaattcagggtctgacttgcagccaact

SEQ ID NO: 98 - DNA, 40 bp, Homo sapiens
caagtccatctctaattcaggcaaggccaggccccagccc

SEQ ID NO: 99 - DNA, 40 bp, Homo sapiens
caagatagatattatagcaggtggcttttgttttacagaa

SEQ ID NO: 100 - DNA, 40 bp, Homo sapiens
caagatagatattatagcagaacttcgatatgacctgcca

SEQ ID NO: 101 - DNA, 40 bp, Homo sapiens
gaaaccaactaaaggcaaagcccattttccttctttcgca

SEQ ID NO: 102 - DNA, 40 bp, Homo sapiens
gaaaccaactaaaggcaaaggtaaaaaacatgaagcagat

SEQ ID NO: 103 - DNA, 40 bp, Homo sapiens
ggggacagtgaaatttggtggcaagaatgaggtgacactg

SEQ ID NO: 104 - DNA, 40 bp, Homo sapiens
ggggacagtgaaatttggtgggcagctgctttcctttgac

SEQ ID NO: 105 - DNA, 40 bp, Homo sapiens
ctcagagccaggctgtagagatgttttctacctttccaca

SEQ ID NO: 106 - DNA, 40 bp, Homo sapiens
ctcagagccaggctgtagagtccgctctatcaagctgaag

SEQ ID NO: 107 - DNA, 40 bp, Homo sapiens
gaggagccacactctgacagatacctggctgagagctggc

SEQ ID NO: 108 - DNA, 40 bp, Homo sapiens
gaggagccacactctgacagtgagggtgcggggtcaggcg

SEQ ID NO: 109 - DNA, 40 bp, Homo sapiens
actcgcgcctcttccatctgttttgtcgcagccggaatac

SEQ ID NO: 110 - DNA, 40 bp, Homo sapiens
actcgcgcctcttccatctgccggaatacacctggcgtct

SEQ ID NO: 111 - DNA, 40 bp, Homo sapiens
acttccttagtggtttccaggttgccagggcactgcagct

SEQ ID NO: 112 - DNA, 40 bp, Homo sapiens
acttccttagtggtttccaggtggtggtgctcaccaacac

SEQ ID NO: 113 - DNA, 40 bp, Homo sapiens
gtcttgagaattggaagcaggtggtggtgctcaccaacac

SEQ ID NO: 114 - DNA, 40 bp, Homo sapiens
tccagagcccacagtcccagctgcaccttacctgctcccc

SEQ ID NO: 115 - DNA, 40 bp, Homo sapiens
tccagagcccacagtcccaggggtccatgatgccgagctg

SEQ ID NO: 116 - DNA, 40 bp, Homo sapiens
ccaagttttgtgaaagaaagtgtatgttttgttcacgaca

SEQ ID NO: 117 - DNA, 40 bp, Homo sapiens
ccaagttttgtgaaagaaagaacatcagataccaaaccta

SEQ ID NO: 118 - DNA, 40 bp, Homo sapiens
tcttcacagaacacactcaagtgcttgtaggtcttggtgc

SEQ ID NO: 119 - DNA, 40 bp, Homo sapiens
tcttcacagaacacactcaaccccctgcctgggatgcgcc

SEQ ID NO: 120 - DNA, 40 bp, Homo sapiens
gagaagctcacgattaccaggcacctcattgtgaacatgc

SEQ ID NO: 121 - DNA, 40 bp, Homo sapiens
tcttggaggagccagtacaggcacctcattgtgaacatgc

SEQ ID NO: 122 - DNA, 40 bp, Homo sapiens
gtggggggccattgctgcattttgtattttccaggtacag

SEQ ID NO: 123 - DNA, 40 bp, Homo sapiens
gtggggggccattgctgcatgtacagtctttgcccgctgc

SEQ ID NO: 124 - DNA, 40 bp, Homo sapiens
tactgaaatgtgatgaacatatccaggtaatcgagagacc

SEQ ID NO: 125 - DNA, 40 bp, Homo sapiens
tactgaaatgtgatgaacatatccagaagcttggaagctg

SEQ ID NO: 126 - DNA, 40 bp, Homo sapiens
gaatctcttatcattgatggttcctgttcagattgtgatg

SEQ ID NO: 127 - DNA, 40 bp, Homo sapiens
gaatctcttatcattgatggtttatttatggagattctta

SEQ ID NO: 128 - DNA, 40 bp, Homo sapiens
ctccatgctcagctctctggtttctttcagggcctgccat

SEQ ID NO: 129 - DNA, 40 bp, Homo sapiens
ctccatgctcagctctctggggaaggtgaagaaggagctg

SEQ ID NO: 130 - DNA, 40 bp, Homo sapiens
cttggagctgacgccgacggggaactgacaagatcacatt

SEQ ID NO: 131 - DNA, 40 bp, Homo sapiens
cttggagctgacgccgacggtttattgcagggaactgaca

SEQ ID NO: 132 - DNA, 40 bp, Homo sapiens
tccagcctgggcgacagaagtcttgtctcaagaagaaaac

SEQ ID NO: 133 - DNA, 40 bp, Homo sapiens
ctatcaaaagaggatatgtttcttgtctcaagaagaaaac

SEQ ID NO: 134 - DNA, 40 bp, Homo sapiens
tgcggagcaagagtggacatcgtttgtttcccatttctcc

SEQ ID NO: 135 - DNA, 40 bp, Homo sapiens
tgcggagcaagagtggacataaactttacattttcctgtt

SEQ ID NO: 136 - DNA, 40 bp, Homo sapiens
agtccagccccagcatggcacctctccccactcctaggtc

SEQ ID NO: 137 - DNA, 40 bp, Homo sapiens
agtccagccccagcatggcagtcctgtacatccaggcctt

SEQ ID NO: 138 - DNA, 40 bp, Homo sapiens
caagcaggtccaaagagagattttggtaaacagagctcca

SEQ ID NO: 139 - DNA, 40 bp, Homo sapiens
caagcaggtccaaagagagaagctccaagagtcaggatcg

SEQ ID NO: 140 - DNA, 40 bp, Homo sapiens
ctctctccaacctgcattctcatctcgcccacagttggat

SEQ ID NO: 141 - DNA, 40 bp, Homo sapiens
ctctctccaacctgcattctttggatcgatcaacccggga

SEQ ID NO: 142 - DNA, 40 bp, Homo sapiens
caccacgccgaggccacgagacattgatggaagcagaaac

SEQ ID NO: 143 - DNA, 40 bp, Homo sapiens
caccacgccgaggccacgagtatttcatagacattgatgg

SEQ ID NO: 144 - DNA, 40 bp, Homo sapiens
gcctcactgagcaaccaagagtagtgacttgtcaggagga

SEQ ID NO: 145 - DNA, 40 bp, Homo sapiens
gcctcactgagcaaccaagagtgtcagttgtacccgaggc

SEQ ID NO: 146 - DNA, 40 bp, Homo sapiens
gggagatggataccgacttgctcaatttcagtgatcaacg

SEQ ID NO: 147 - DNA, 40 bp, Homo sapiens
gggagatggataccgacttgtgatcaacgatgggaagctg

SEQ ID NO: 148 - DNA, 40 bp, Homo sapiens
aggatgtggctggcacagaagtgtcatcaggtccctgcag

SEQ ID NO: 149 - DNA, 40 bp, Homo sapiens
aggatgtggctggcacagaaatgagtcagtctgacagtgg

SEQ ID NO: 150 - DNA, 40 bp, Homo sapiens
ttctccaggaccttgccagaccttttctatagggaatcaa

SEQ ID NO: 151 - DNA, 40 bp, Homo sapiens
ttctccaggaccttgccagaggaatcaaagactccatctg

SEQ ID NO: 152 - DNA, 40 bp, Homo sapiens
agctgaaatttccagtaaaggggggttttattcttctttt

SEQ ID NO: 153 - DNA, 40 bp, Homo sapiens
agctgaaatttccagtaaagcctggagatttgaaaaagag

SEQ ID NO: 154 - DNA, 40 bp, Homo sapiens
gatgtcactgtgactatcaagggccgtctttcttctaggt

SEQ ID NO: 155 - DNA, 40 bp, Homo sapiens
gatgtcactgtgactatcaagtcttccatcgacagtgaac

SEQ ID NO: 156 - DNA, 40 bp, Homo sapiens
tatccattcctgagttacagtataaacttccttctcatgc

SEQ ID NO: 157 - DNA, 40 bp, Homo sapiens
tatccattcctgagttacagtgtcttaatattgaaaatga

SEQ ID NO: 158 - DNA, 40 bp, Homo sapiens
tacaagagctgggtggagagggtcccaacaggtattatcg

SEQ ID NO: 159 - DNA, 40 bp, Homo sapiens
tacaagagctgggtggagaggtattatcgagacattgcaa

SEQ ID NO: 160 - DNA, 40 bp, Homo sapiens
agccatttatttgtcccgtgggaaccaatctgcccttttg

SEQ ID NO: 161 - DNA, 40 bp, Homo sapiens
agccatttatttgtcccgtgggtttttttccagggaacca

SEQ ID NO: 162 - DNA, 40 bp, Homo sapiens
agttacaacgaacacctcagtgactcttttacaggaggca

SEQ ID NO: 163 - DNA, 40 bp, Homo sapiens
agttacaacgaacacctcaggaggcaataacagatggctt

SEQ ID NO: 164 - DNA, 40 bp, Homo sapiens
tcacacaggataatttgaaagtgtcagttgtacccgaggc

SEQ ID NO: 165 - DNA, 40 bp, Homo sapiens
cggcgcgggcaacctggcggcccccatttcaggtctgaag

SEQ ID NO: 166 - DNA, 40 bp, Homo sapiens
cggcgcgggcaacctggcgggtctgaaggggcgtctcgat

SEQ ID NO: 167 - DNA, 40 bp, Homo sapiens
ccaccgccatcgacgtgcagtacctctttttaccaccagg

SEQ ID NO: 168 - DNA, 40 bp, Homo sapiens
ccaccgccatcgacgtgcaggtggggctcctgtacgaaga

SEQ ID NO: 169 - DNA, 40 bp, Homo sapiens
ctatgggctcactcctctggtcctcctgttgcagttcgtc

SEQ ID NO: 170 - DNA, 40 bp, Homo sapiens
ctatgggctcactcctctggttcgtcgcctgcagcttcga

SEQ ID NO: 171 - DNA, 40 bp, Homo sapiens
tatctctgggaaaaaacacatttctttttttgcaggggac

SEQ ID NO: 172 - DNA, 40 bp, Homo sapiens
tatctctgggaaaaaacacagggacctgatggggtgcagc

SEQ ID NO: 173 - DNA, 40 bp, Homo sapiens
tcatccagagcccagagcaggggatgtctgaccagatgca

SEQ ID NO: 174 - DNA, 40 bp, Homo sapiens
tcatccagagcccagagcagatgcaagtgctgctggacca

SEQ ID NO: 175 - DNA, 40 bp, Homo sapiens
ccaaggactgcactgtgaaggcccccgccccgcgacctgg

SEQ ID NO: 176 - DNA, 40 bp, Homo sapiens
ccaaggactgcactgtgaagatctggagcaacgacctgac

SEQ ID NO: 177 - DNA, 40 bp, Homo sapiens
cccgagctcagagagtaaattctccttacagacactgaaa

SEQ ID NO: 178 - DNA, 40 bp, Homo sapiens
cccgagctcagagagtaaatatgagatcgcctctgtccca

SEQ ID NO: 179 - DNA, 40 bp, Homo sapiens
gtgcttggagccctgtgcagactttccgcagggtgtgcgc

SEQ ID NO: 180 - DNA, 40 bp, Homo sapiens
gtgcttggagccctgtgcagcctggtgacagactttccgc

SEQ ID NO: 181 - DNA, 40 bp, Homo sapiens
gctggacacgctgaccaaggcatcacttaggagctgctac

SEQ ID NO: 182 - DNA, 40 bp, Homo sapiens
gctggacacgctgaccaaggtgttggtagccttatatgaa

SEQ ID NO: 183 - DNA, 40 bp, Homo sapiens
cccctgagatgaagaaagagctccctgttgacagctgcct

SEQ ID NO: 184 - DNA, 40 bp, Homo sapiens
cccctgagatgaagaaagagctcctgagcagcctgactga

SEQ ID NO: 185 - DNA, 40 bp, Homo sapiens
ctgaactttgggcctgaatgatgtgtttggaccccgaata

SEQ ID NO: 186 - DNA, 40 bp, Homo sapiens
ctgaactttgggcctgaatggctccgagctctgtccagtg

SEQ ID NO: 187 - DNA, 40 bp, Homo sapiens
agatcgcctggctcagtcagtttttctctctagacatggc

SEQ ID NO: 188 - DNA, 40 bp, Homo sapiens
agatcgcctggctcagtcagacatggccaaacgtgtagcc

SEQ ID NO: 189 - DNA, 40 bp, Homo sapiens
ggaggtggacctgagtgaacaatttctcccctctttttag

SEQ ID NO: 190 - DNA, 40 bp, Homo sapiens
ggaggtggacctgagtgaaccacccaactggtcagctaac

SEQ ID NO: 191 - DNA, 40 bp, Homo sapiens
tacagatggtaaaatgcaagtttgatttttcatatccagg

SEQ ID NO: 192 - DNA, 40 bp, Homo sapiens
tacagatggtaaaatgcaaggaattgccacaagcagtctg

SEQ ID NO: 193 - DNA, 40 bp, Homo sapiens
ccctgctcatcacctacgggtctgtcccaggctctctggg

SEQ ID NO: 194 - DNA, 40 bp, Homo sapiens
ccctgctcatcacctacgggccctatgccatcaatgggaa

SEQ ID NO: 195 - DNA, 40 bp, Homo sapiens
ggctcccattctggttaaagagtgttctcatttccaatag

SEQ ID NO: 196 - DNA, 40 bp, Homo sapiens
ggctcccattctggttaaaggccagtctgccatccatcca

SEQ ID NO: 197 - DNA, 40 bp, Homo sapiens
ctgcacttataaatattcagtgttccaccttgcagacccg

SEQ ID NO: 198 - DNA, 40 bp, Homo sapiens
ctgcacttataaatattcagacccgaggggaagctgcagc

SEQ ID NO: 199 - DNA, 40 bp, Homo sapiens
cgctggcaccatgaacccagtatttccaggaccaagtgag

SEQ ID NO: 200 - DNA, 40 bp, Homo sapiens
cgctggcaccatgaacccagagagcagtatctttattgag

SEQ ID NO: 201 - DNA, 40 bp, Homo sapiens
ccctagtctgattcctttaggttggtgtaatcagctgggg

SEQ ID NO: 202 - DNA, 40 bp, Homo sapiens
ttccccatcaacatcaaaagttttgttgtctgcagttcca

SEQ ID NO: 203 - DNA, 40 bp, Homo sapiens
ttccccatcaacatcaaaagttccaatggtggcagtaaga

SEQ ID NO: 204 - DNA, 40 bp, Homo sapiens
ccagctgcattgcaagttcggactgtgagtccctgcaggc

SEQ ID NO: 205 - DNA, 40 bp, Homo sapiens
ccagctgcattgcaagttcggggtgcggaagactcacaac

SEQ ID NO: 206 - DNA, 40 bp, Homo sapiens
ggccagcccccttctccacggccttgcccactaggtaacc

SEQ ID NO: 207 - DNA, 40 bp, Homo sapiens
ggccagcccccttctccacggtaaccatgtgcgaccgaaa

SEQ ID NO: 208 - DNA, 40 bp, Homo sapiens
cgctctccgccttccagaaggggtctccttatgccaggga

SEQ ID NO: 209 - DNA, 40 bp, Homo sapiens
agggagacgttccctgcctggggtctccttatgccaggga

SEQ ID NO: 210 - DNA, 40 bp, Homo sapiens
ttggaagcgaatcccccaagtcctttgttcttttgcagtg

SEQ ID NO: 211 - DNA, 40 bp, Homo sapiens
ttggaagcgaatcccccaagtgatgtatatctctcatcaa

SEQ ID NO: 212 - DNA, 40 bp, Homo sapiens
ctacggcggtgccctcctcacccccttttcatcccccgcc

SEQ ID NO: 213 - DNA, 40 bp, Homo sapiens
ctacggcggtgccctcctcagcatctccctgatcatgtgg

SEQ ID NO: 214 - DNA, 40 bp, Homo sapiens
cctggtcgcagttcaacaagatgaggaatctgatgctcag

SEQ ID NO: 215 - DNA, 40 bp, Homo sapiens
cctggtcgcagttcaacaaggagatcctgctgggccgtgg

SEQ ID NO: 216 - DNA, 40 bp, Homo sapiens
caccaagcagaggcttccagtctgtctgccctttctgtag

SEQ ID NO: 217 - DNA, 40 bp, Homo sapiens
caccaagcagaggcttccaggccagaagccttttaaaagg

SEQ ID NO: 218 - DNA, 40 bp, Homo sapiens
gggactcccccaaagacaagcttttctttcagtaaatgta

SEQ ID NO: 219 - DNA, 40 bp, Homo sapiens
gggactcccccaaagacaaggtcccattttcagtgcccaa

SEQ ID NO: 220 - DNA, 40 bp, Homo sapiens
gcactgctgttcaacctcggcttctcccttcctctcaccc

SEQ ID NO: 221 - DNA, 40 bp, Homo sapiens
gcactgctgttcaacctcgggggcaagtatagcgcatttg

SEQ ID NO: 222 - DNA, 40 bp, Homo sapiens
acgagaccattgccttcaaggagccctctctgtcccccgc

SEQ ID NO: 223 - DNA, 40 bp, Homo sapiens
acgagaccattgccttcaaggtgccgagcagagagatcga

SEQ ID NO: 224 - DNA, 40 bp, Homo sapiens
aagatgtccctgtgaggattgtgtgtttgtttccacaggc

SEQ ID NO: 225 - DNA, 40 bp, Homo sapiens
aagatgtccctgtgaggattgcactgggtgcaagttcctg

SEQ ID NO: 226 - DNA, 40 bp, Homo sapiens
agagaagtcgtttcattcaatctgattcctttaggtcagc

SEQ ID NO: 227 - DNA, 40 bp, Homo sapiens
agcccagcagttccgaaatgtctcccttctccagcgcccc

SEQ ID NO: 228 - DNA, 40 bp, Homo sapiens
agcccagcagttccgaaatgcgcccccattcctggaggac

SEQ ID NO: 229 - DNA, 40 bp, Homo sapiens
ccctcccccggctcctgtcggcctgggcagcatggccgta

SEQ ID NO: 230 - DNA, 40 bp, Homo sapiens
tgattccaagcaaaaaccagccttcccctaggtcttcaga

SEQ ID NO: 231 - DNA, 40 bp, Homo sapiens
tgattccaagcaaaaaccaggctccatctactctttgaag

SEQ ID NO: 232 - DNA, 40 bp, Homo sapiens
caagtccatctctaattcagccaactctcaaggcaaggcc

SEQ ID NO: 233 - DNA, 40 bp, Homo sapiens
ctatcaaaagaggatatgttcattttaggaggccaaggca

SEQ ID NO: 234 - DNA, 40 bp, Homo sapiens
gtcttccaatggcccctcagccttttctctaggaaatgat

SEQ ID NO: 235 - DNA, 40 bp, Homo sapiens
gtcttccaatggcccctcaggaaatgatacacctgaagaa

SEQ ID NO: 236 - DNA, 40 bp, Homo sapiens
gcacctccccgggacgcctgcccttgtctggaaagaagtt

SEQ ID NO: 237 - DNA, 40 bp, Homo sapiens
gcacctccccgggacgcctgtcaccggactttgctgagga

SEQ ID NO: 238 - DNA, 40 bp, Homo sapiens
tggaccccagaccacaccggaagaaatgagccagaagtga

SEQ ID NO: 239 - DNA, 40 bp, Homo sapiens
gtcccggaaccacatgcacgaagaaatgagccagaagtga

SEQ ID NO: 240 - DNA, 40 bp, Homo sapiens
tctgtgttcccatcgcacaggaatcctacgccaacgtgaa

SEQ ID NO: 241 - DNA, 40 bp, Homo sapiens
tgtatgacgtcactgaccaggaatcctacgccaacgtgaa

SEQ ID NO: 242 - DNA, 40 bp, Homo sapiens
ggaatatgatcccaccctcgtacttctcaaagaggatggc

SEQ ID NO: 243 - DNA, 40 bp, Homo sapiens
ggaatatgatcccaccctcgaatcaacctaccgacaccaa

SEQ ID NO: 244 - DNA, 40 bp, Homo sapiens
gaactggcaccgacagacagtgtcccctccctccccagat

SEQ ID NO: 245 - DNA, 40 bp, Homo sapiens
gaactggcaccgacagacagatcctgtttctggaccttgg

SEQ ID NO: 246 - DNA, 40 bp, Homo sapiens
tgatgaagacctttccccagatctcttaggtgaagacatg

SEQ ID NO: 247 - DNA, 40 bp, Homo sapiens
tgatgaagacctttccccaggccccgagcattcctctgat

SEQ ID NO: 248 - DNA, 40 bp, Homo sapiens
ccaggccgacatggagagcagccccacccacaggcaagga

SEQ ID NO: 249 - DNA, 40 bp, Homo sapiens
ccaggccgacatggagagcagcaaggagcccggcctgttt

SEQ ID NO: 250 - DNA, 40 bp, Homo sapiens
acatgaaggtggacggagagttctctgtgaccagacatga

SEQ ID NO: 251 - DNA, 40 bp, Homo sapiens
ttcgtccatatgtgcataagcttcttctcttttctctttt

SEQ ID NO: 252 - DNA, 40 bp, Homo sapiens
ttcgtccatatgtgcataagatcctcgtggtcattgaacc

SEQ ID NO: 253 - DNA, 40 bp, Homo sapiens
agggatggccagtggtagtgggtctccaactgaattcctt

SEQ ID NO: 254 - DNA, 40 bp, Homo sapiens
agaagggagcgatactacagggtctccaactgaattcctt

SEQ ID NO: 255 - DNA, 40 bp, Homo sapiens
ccaatgtggttcaaaacacattatctcatctgcagggtaa

SEQ ID NO: 256 - DNA, 40 bp, Homo sapiens
ccaatgtggttcaaaacacaggtaaaagtgtcttaactgg

SEQ ID NO: 257 - DNA, 40 bp, Homo sapiens
ccattgatgcaaacgcagcaatggagtttcgctcctgttg

SEQ ID NO: 258 - DNA, 40 bp, Homo sapiens
ccattgatgcaaacgcagcagaacttgccacatcagactc

SEQ ID NO: 259 - DNA, 40 bp, Homo sapiens
gctgcatctggaggtcctgggaagcagaatctggtaatat

SEQ ID NO: 260 - DNA, 40 bp, Homo sapiens
cagtgttagtgaatgactatgaagcagaatctggtaatat

SEQ ID NO: 261 - DNA, 40 bp, Homo sapiens
acaaggacacagaaaacaagccttcccacacaggccctgc

SEQ ID NO: 262 - DNA, 40 bp, Homo sapiens
acaaggacacagaaaacaagctggagcaccgctgcacctc

SEQ ID NO: 263 - DNA, 40 bp, Homo sapiens
agctcggaccaagcgctcagttttaaaattgctatagctt

SEQ ID NO: 264 - DNA, 40 bp, Homo sapiens
agctcggaccaagcgctcagcttagcctgcgacgcttatg

SEQ ID NO: 265 - DNA, 40 bp, Homo sapiens
agggggctctttatataatgtttgtgcctttctttcgcag

SEQ ID NO: 266 - DNA, 40 bp, Homo sapiens
agggggctctttatataatgtgctgcatggtgctgaacca

SEQ ID NO: 267 - DNA, 40 bp, Homo sapiens
gcccccaactgagaagctgggctggagtgctgtggcacaa

SEQ ID NO: 268 - DNA, 40 bp, Homo sapiens
gcccccaactgagaagctggtgcccttggtgtggtggaag

SEQ ID NO: 269 - DNA, 40 bp, Homo sapiens
gaacgagatctcatcccactaactacaaagagctggagct

SEQ ID NO: 270 - DNA, 40 bp, Homo sapiens
agtatcagaaggacaaaaagaactacaaagagctggagct

SEQ ID NO: 271 - DNA, 40 bp, Homo sapiens
tgaaggtccagggcatggagcctgtctcctggcagtgtct

SEQ ID NO: 272 - DNA, 40 bp, Homo sapiens
tgaaggtccagggcatggagtgtctctatggctgctacgt

SEQ ID NO: 273 - DNA, 40 bp, Homo sapiens
ggcggccgcgccggctccaggaaatggcaactgctgacag

SEQ ID NO: 274 - DNA, 40 bp, Homo sapiens
ggcggccgcgccggctccagggccatgaagcccccaggag

SEQ ID NO: 275 - DNA, 40 bp, Homo sapiens
ccttccagctacatcgaaacgcatgaggatgttgtatttc

SEQ ID NO: 276 - DNA, 40 bp, Homo sapiens
ccttccagctacatcgaaactttacctaaagcagtaaaaa

SEQ ID NO: 277 - DNA, 40 bp, Homo sapiens
cttttctcttctttttataggttgaacaaatcctggcaga

SEQ ID NO: 278 - DNA, 40 bp, Homo sapiens
gatgtgatgaactatcttcggttgaacaaatcctggcaga

SEQ ID NO: 279 - DNA, 40 bp, Homo sapiens
gcactgggcattcagaaaagtctctcttcctcacccctgc

SEQ ID NO: 280 - DNA, 40 bp, Homo sapiens
gcactgggcattcagaaaaggttctccccggaggtgctgg

SEQ ID NO: 281 - DNA, 40 bp, Homo sapiens
ctgtcacaggggagtttacgtcttgcatgtctctcttaca

SEQ ID NO: 282 - DNA, 40 bp, Homo sapiens
ctgtcacaggggagtttacgggaatgccagagcagtgggc

SEQ ID NO: 283 - DNA, 40 bp, Homo sapiens
gggtgcaaaagatcctgcagccattccaggttgctgaggt

SEQ ID NO: 284 - DNA, 40 bp, Homo sapiens
gggtgcaaaagatcctgcaggactacaaatccctccagga

SEQ ID NO: 285 - DNA, 40 bp, Homo sapiens
ggcaccccaaaagatggcagatcagtctctccctgttctc

SEQ ID NO: 286 - DNA, 40 bp, Homo sapiens
ggcaccccaaaagatggcaggtgcgagcccgaccaaggat

SEQ ID NO: 287 - DNA, 40 bp, Homo sapiens
gcatctcagcccaagagaagtttctttgcaggttatattc

SEQ ID NO: 288 - DNA, 40 bp, Homo sapiens
gcatctcagcccaagagaaggttatattcccagaggatgt

SEQ ID NO: 289 - DNA, 40 bp, Homo sapiens
cttgccttcccatcctcctgcaaacacctgccacctttct

SEQ ID NO: 290 - DNA, 40 bp, Homo sapiens
cttgccttcccatcctcctgaacttccaggtcctgagtca

SEQ ID NO: 291 - DNA, 40 bp, Homo sapiens
ctacacagagctgcagcaaggtgtgcacccagctgcaggt

SEQ ID NO: 292 - DNA, 40 bp, Homo sapiens
ctacacagagctgcagcaagctctgtcccaaatgggctac

SEQ ID NO: 293 - DNA, 40 bp, Homo sapiens
acctgttaccactttcaaaatttctgtgctaaacagtgtt

SEQ ID NO: 294 - DNA, 40 bp, Homo sapiens
acctgttaccactttcaaaaatctacagacagtcaatgtg

SEQ ID NO: 295 - DNA, 40 bp, Homo sapiens
agacaagggattggtggaaacattttattttacagaattg

SEQ ID NO: 296 - DNA, 40 bp, Homo sapiens
agacaagggattggtggaaaaattgacagcgtatgccatg

SEQ ID NO: 297 - DNA, 40 bp, Homo sapiens
caacgagaacaagctatcagttacttttaccccacagggc

SEQ ID NO: 298 - DNA, 40 bp, Homo sapiens
caacgagaacaagctatcagggctgctaaggaagcaaaaa

SEQ ID NO: 299 - DNA, 40 bp, Homo sapiens
tctatatcccctctaagacgcacttctttcccctctgtag

SEQ ID NO: 300 - DNA, 40 bp, Homo sapiens
tctatatcccctctaagacggacctgggtgcagccgcagg

SEQ ID NO: 301 - DNA, 40 bp, Homo sapiens
tggagccagttactgggcaggtgtgtttttgtgacagtca

SEQ ID NO: 302 - DNA, 40 bp, Homo sapiens
tggagccagttactgggcaggtgtctgtactggtgatgtg

SEQ ID NO: 303 - DNA, 40 bp, Homo sapiens
aaaagaaactgaggaatcagtatcacaggcagaagctctg

SEQ ID NO: 304 - DNA, 40 bp, Homo sapiens
aaaagaaactgaggaatcagccttagtatcacaggcagaa

SEQ ID NO: 305 - DNA, 40 bp, Homo sapiens
cagcactaggttataaagaggagtctagtaaaagccctaa

SEQ ID NO: 306 - DNA, 40 bp, Homo sapiens
cagcactaggttataaagagaggatgtcttatatcttaaa

SEQ ID NO: 307 - DNA, 40 bp, Homo sapiens
gcccccgttttcctgcccagcccttgtcctcagtgcaccc

SEQ ID NO: 308 - DNA, 40 bp, Homo sapiens
gcccccgttttcctgcccagtacctgaagctgcgggagcg

SEQ ID NO: 309 - DNA, 40 bp, Homo sapiens
gccgccgccgccgccgccaggctctgatgctggtgtctgg

SEQ ID NO: 310 - DNA, 40 bp, Homo sapiens
caccttatgaagtatagcaggctctgatgctggtgtctgg

SEQ ID NO: 311 - DNA, 40 bp, Homo sapiens
agtggcagtggctgtaccagcccacaggaaacaacccgta

SEQ ID NO: 312 - DNA, 40 bp, Homo sapiens
agtggcagtggctgtaccagctcttggtggagggctccac

SEQ ID NO: 313 - DNA, 40 bp, Homo sapiens
gagattctgaagataaggagttctcttgtaggatgccact

SEQ ID NO: 314 - DNA, 40 bp, Homo sapiens
gagattctgaagataaggaggtaaaacctgtttagaaatt

SEQ ID NO: 315 - DNA, 40 bp, Homo sapiens
ccaagagacagcacattcagctcctgagcagcctgactga

SEQ ID NO: 316 - DNA, 40 bp, Homo sapiens
tcagagcagtcgggacacaggacacctgactgatagtgaa

SEQ ID NO: 317 - DNA, 40 bp, Homo sapiens
ctacgacagtgaagattcaggacacctgactgatagtgaa

SEQ ID NO: 318 - DNA, 40 bp, Homo sapiens
ctgttgtgtccgttttgaagagccctttgctcctccctca

SEQ ID NO: 319 - DNA, 40 bp, Homo sapiens
ctgttgtgtccgttttgaagaatgaacggagaccagaatt

SEQ ID NO: 320 - DNA, 40 bp, Homo sapiens
ccggccctacaggctggcggataaacccactgccctacag

SEQ ID NO: 321 - DNA, 40 bp, Homo sapiens
ccctccgcctcctgatgcagataaacccactgccctacag

SEQ ID NO: 322 - DNA, 40 bp, Homo sapiens
gagattctgaagataaggaggatgccactggaaatgttga

SEQ ID NO: 323 - DNA, 40 bp, Homo sapiens
tgaaaagtccagaggaagaggttgtggcagcactgcctga

SEQ ID NO: 324 - DNA, 40 bp, Homo sapiens
tcctggaggagctacgcagggttgtggcagcactgcctga

SEQ ID NO: 325 - DNA, 40 bp, Homo sapiens
gtcatggcagaagacctccatccaagacatctctggcatc

SEQ ID NO: 326 - DNA, 40 bp, Homo sapiens
ctatagctactggatatgggtccaagacatctctggcatc

SEQ ID NO: 327 - DNA, 40 bp, Homo sapiens
ccggagccccttcaaaaaagacttttcgtgttttacagtc

SEQ ID NO: 328 - DNA, 40 bp, Homo sapiens
ccggagccccttcaaaaaagtctgttgccagaatcggcca

SEQ ID NO: 329 - DNA, 40 bp, Homo sapiens
ccacagatactattaggaggccataccaccctgaacgcgc

SEQ ID NO: 330 - DNA, 40 bp, Homo sapiens
ccacagatactattaggagggaatttatcatggcatccag

SEQ ID NO: 331 - DNA, 40 bp, Homo sapiens
tgttcaagttcccaaagcaggagatcctgctgggccgtgg

SEQ ID NO: 332 - DNA, 40 bp, Homo sapiens
actcccagctcaatgcaatggttccataccatctggtact

SEQ ID NO: 333 - DNA, 40 bp, Homo sapiens
actcccagctcaatgcaatggctcatcagattcaagagat

SEQ ID NO: 334 - DNA, 40 bp, Homo sapiens
atcactgtgacttccctgaggtctctgctcctcagctgct

SEQ ID NO: 335 - DNA, 40 bp, Homo sapiens
atcactgtgacttccctgagctgctgtcccccagcaacgt

SEQ ID NO: 336 - DNA, 40 bp, Homo sapiens
atcctctcaatcaaaataagtttgtgtgcacttttctgct

SEQ ID NO: 337 - DNA, 40 bp, Homo sapiens
atcctctcaatcaaaataagggtaaaccagacttgaatac

SEQ ID NO: 338 - DNA, 40 bp, Homo sapiens
ctattcctttattgaatttgttttcttcatcattctagat

SEQ ID NO: 339 - DNA, 40 bp, Homo sapiens
ctattcctttattgaatttgatactttcattcagaaaacc

SEQ ID NO: 340 - DNA, 40 bp, Homo sapiens
agtcatacctggagcagcagtttgtttcttttctagaaaa

SEQ ID NO: 341 - DNA, 40 bp, Homo sapiens
agtcatacctggagcagcagaaaaaattgaaagaactgtc

SEQ ID NO: 342 - DNA, 40 bp, Homo sapiens
gcaaccagtttgggcatcagctgcccttctctcctgtagg

SEQ ID NO: 343 - DNA, 40 bp, Homo sapiens
gcaaccagtttgggcatcaggagaacgccaagaacgaaga

SEQ ID NO: 344 - DNA, 40 bp, Homo sapiens
ccatggtcaaaaaatggcagcaccaacaggtccgccaaat

SEQ ID NO: 345 - DNA, 40 bp, Homo sapiens
ccatggtcaaaaaatggcagacaatgattgaagctcacgt

SEQ ID NO: 346 - DNA, 40 bp, Homo sapiens
gcctgatgcccgaatttcaggccatgaagtacttgtcata

SEQ ID NO: 347 - DNA, 40 bp, Homo sapiens
gcctgatgcccgaatttcagtttggcacttacagcgaatc

SEQ ID NO: 348 - DNA, 40 bp, Homo sapiens
agattgaagctaaaattaagttttctgtcttacccattcc

SEQ ID NO: 349 - DNA, 40 bp, Homo sapiens
agattgaagctaaaattaaggagctgacaagtacttgtag

SEQ ID NO: 350 - DNA, 40 bp, Homo sapiens
agcacaagctatgtatcaagcataactttcttctacagga

SEQ ID NO: 351 - DNA, 40 bp, Homo sapiens
agcacaagctatgtatcaaggattctggagtgaagcagat

SEQ ID NO: 352 - DNA, 40 bp, Homo sapiens
agatgtaaaagtgtcactgttttggttttcagttacagct

SEQ ID NO: 353 - DNA, 40 bp, Homo sapiens
agatgtaaaagtgtcactgtttacagctttcttcctggct

SEQ ID NO: 354 - DNA, 40 bp, Homo sapiens
ctgcagcctccgcctcccaggaacttgccacatcagactc

SEQ ID NO: 355 - DNA, 40 bp, Homo sapiens
aggatgatgcagcatccaactggtctttttgtgttctgtg

SEQ ID NO: 356 - DNA, 40 bp, Homo sapiens
aggatgatgcagcatccaacgcgggcacatgaacgccccc

SEQ ID NO: 357 - DNA, 40 bp, Homo sapiens
tggtgaaatggaccccaaagtctttctctttcaagtacct

SEQ ID NO: 358 - DNA, 40 bp, Homo sapiens
tggtgaaatggaccccaaagtacctgctattgaggagaac

SEQ ID NO: 359 - DNA, 40 bp, Homo sapiens
agcttaaagaactgtattcgtttgactgcaaccctggagt

SEQ ID NO: 360 - DNA, 40 bp, Homo sapiens
gatcaaggcaaccgggaaagtttgactgcaaccctggagt

SEQ ID NO: 361 - DNA, 40 bp, Homo sapiens
aacacaccaactttgtggaggtcctggcaatctccgttgc

SEQ ID NO: 362 - DNA, 40 bp, Homo sapiens
aacacaccaactttgtggagttccggaactttaagatcat

SEQ ID NO: 363 - DNA, 40 bp, Homo sapiens
gcgggtctgcagcctacgcaaactgaagcaggcccagacc

SEQ ID NO: 364 - DNA, 40 bp, Homo sapiens
gttccaggtcctcctggcagaactgaagcaggcccagacc

SEQ ID NO: 365 - DNA, 40 bp, Homo sapiens
cccgctgccccagctcaaagatcagtgctaacatcttccg

SEQ ID NO: 366 - DNA, 40 bp, Homo sapiens
attctgatatagtaaaaatgatcagtgctaacatcttccg

SEQ ID NO: 367 - DNA, 40 bp, Homo sapiens
atgagtttcccaccgatggggaggaagaccgcaggaagga

SEQ ID NO: 368 - DNA, 40 bp, Homo sapiens
atgagtttcccaccgatggggagatgtcagcgcaggagga

SEQ ID NO: 369 - DNA, 40 bp, Homo sapiens
agtttatttaacatttgatgagcctaccttgtacaatgct

SEQ ID NO: 370 - DNA, 40 bp, Homo sapiens
agtttatttaacatttgatgaacttcgagaaaccaagacc

SEQ ID NO: 371 - DNA, 40 bp, Homo sapiens
ccacctagcagccaccagagaccagaggtggcacaggcag

SEQ ID NO: 372 - DNA, 40 bp, Homo sapiens
ccacctagcagccaccagaggttacaaggggagagtggcc

SEQ ID NO: 373 - DNA, 40 bp, Homo sapiens
tccaggatcctgaggcatggccatatcagcgggaacaaga

SEQ ID NO: 374 - DNA, 40 bp, Homo sapiens
ggcagcggaggggcgacaaaccatatcagcgggaacaaga

SEQ ID NO: 375 - DNA, 40 bp, Homo sapiens
ggcaacttcgttaatatgagctttctactcaacaggtcta

SEQ ID NO: 376 - DNA, 40 bp, Homo sapiens
ggcaacttcgttaatatgaggtctatccaggaaaatggtg

SEQ ID NO: 377 - DNA, 40 bp, Homo sapiens
ggagcctgggcatctcgttgccctgcccgtctccctccca

SEQ ID NO: 378 - DNA, 40 bp, Homo sapiens
ggagcctgggcatctcgttggtggagctggcaacaggaca

SEQ ID NO: 379 - DNA, 40 bp, Homo sapiens
ctggtgtgcttgggagccagggttatcatgaagattaaat

SEQ ID NO: 380 - DNA, 40 bp, Homo sapiens
ctggtgtgcttgggagccagagatcacctcctacaccact

SEQ ID NO: 381 - DNA, 40 bp, Homo sapiens
attggaggagcttctggaaagatgccctcttcgcttccca

SEQ ID NO: 382 - DNA, 40 bp, Homo sapiens
attggaggagcttctggaaagtgctcttgatgatttcgat

SEQ ID NO: 383 - DNA, 40 bp, Homo sapiens
aatgacgtgctgcaccactgggccctgacgcgcggaaagt

SEQ ID NO: 384 - DNA, 40 bp, Homo sapiens
aatgacgtgctgcaccactgccagcgcaagcaggcccggg

SEQ ID NO: 385 - DNA, 40 bp, Homo sapiens
gcctggggtggagagggcagccccccagctaccacaagaa

SEQ ID NO: 386 - DNA, 40 bp, Homo sapiens
gcctggggtggagagggcagtctgggatgtggcattggct

SEQ ID NO: 387 - DNA, 40 bp, Homo sapiens
ggaaatgggacaggaggcagaggatcacaggctttaaaat

SEQ ID NO: 388 - DNA, 40 bp, Homo sapiens
ggaaatgggacaggaggcagcttttctctcaacagaggat

SEQ ID NO: 389 - DNA, 40 bp, Homo sapiens
agaccgactgccagtaataggagattgtgaagacctttga

SEQ ID NO: 390 - DNA, 40 bp, Homo sapiens
agaccgactgccagtaatagagcctgttagtattaatgaa

SEQ ID NO: 391 - DNA, 40 bp, Homo sapiens
tcatgctagccgaggcccagtggcggccagaggagtccga

SEQ ID NO: 392 - DNA, 40 bp, Homo sapiens
tcatgctagccgaggcccaggaaaccactatcagcggcct

SEQ ID NO: 393 - DNA, 40 bp, Homo sapiens
gaaggcagctgagcaaacagttctctcccttgcagctgcc

SEQ ID NO: 394 - DNA, 40 bp, Homo sapiens
gaaggcagctgagcaaacagctgcccgggaacaggcaaag

SEQ ID NO: 395 - DNA, 40 bp, Homo sapiens
gccaacagccaattctacaggtacaacaaataacactgtg

SEQ ID NO: 396 - DNA, 40 bp, Homo sapiens
gccaacagccaattctacagctaaacccacagttcagccc

SEQ ID NO: 397 - DNA, 40 bp, Homo sapiens
cccatcaactgcacccactcccctctgacgtccatcatct

SEQ ID NO: 398 - DNA, 40 bp, Homo sapiens
cccatcaactgcacccactcctgtgtggacctggatgaca

SEQ ID NO: 399 - DNA, 40 bp, Homo sapiens
gcggaaagaattgcatgaagagcgacaacaacacaaccag

SEQ ID NO: 400 - DNA, 40 bp, Homo sapiens
gcggaaagaattgcatgaagtttgccatctcttggagcaa

SEQ ID NO: 401 - DNA, 40 bp, Homo sapiens
tgtgggaattacaattcaagcttatcacacagactttcag

SEQ ID NO: 402 - DNA, 40 bp, Homo sapiens
aagaagggatggcagagaagcttatcacacagactttcag

SEQ ID NO: 403 - DNA, 40 bp, Homo sapiens
cttcctcaagtcgcccaaagctcccccgtttcttctcccc

SEQ ID NO: 404 - DNA, 40 bp, Homo sapiens
cttcctcaagtcgcccaaagacaacgtggacgaccccacg

SEQ ID NO: 405 - DNA, 40 bp, Homo sapiens
tcttcgctggtggcaaactgtatcgtgaagagcgcttccg

SEQ ID NO: 406 - DNA, 40 bp, Homo sapiens
tcttcgctggtggcaaactgcgggtgcatctcgacatcca

SEQ ID NO: 407 - DNA, 40 bp, Homo sapiens
gcaagaagtacaaagtggagtatgtgctttgttgtgacag

SEQ ID NO: 408 - DNA, 40 bp, Homo sapiens
gcaagaagtacaaagtggagtatcctatcatgtacagcac

SEQ ID NO: 409 - DNA, 40 bp, Homo sapiens
tgtaggagcaatgactgttgcattctttttctttaggtat

SEQ ID NO: 410 - DNA, 40 bp, Homo sapiens
tgtaggagcaatgactgttggtatgggctattccatgtat

SEQ ID NO: 411 - DNA, 40 bp, Homo sapiens
ccttcctggatccccctaaggtggtattaaagataatcaa

SEQ ID NO: 412 - DNA, 40 bp, Homo sapiens
aagtgcagatagatggccttgtggtattaaagataatcaa

SEQ ID NO: 413 - DNA, 40 bp, Homo sapiens
caggtctaactcgcttccaggccccagcagatgaacctga

SEQ ID NO: 414 - DNA, 40 bp, Homo sapiens
caggtctaactcgcttccaggctgaagcttcagaaaagga

SEQ ID NO: 415 - DNA, 40 bp, Homo sapiens
cctccccatacctgagctcgatggcggtgggaccccccga

SEQ ID NO: 416 - DNA, 40 bp, Homo sapiens
gcaaaaggatataccaggagcatttatttcaggggtcctc

SEQ ID NO: 417 - DNA, 40 bp, Homo sapiens
gcaaaaggatataccaggaggggtcctcaagattcgagat

SEQ ID NO: 418 - DNA, 40 bp, Homo sapiens
cactccaatttatagattctgattcttcatcatggtgtga

SEQ ID NO: 419 - DNA, 40 bp, Homo sapiens
cactccaatttatagattctttcttaaacacttccagtaa

SEQ ID NO: 420 - DNA, 40 bp, Homo sapiens
tgagagtcttcagttactagtttgtctttcctagatccag

SEQ ID NO: 421 - DNA, 40 bp, Homo sapiens
tgagagtcttcagttactagaggcggatttccctgactga

SEQ ID NO: 422 - DNA, 40 bp, Homo sapiens
ttaacagcattttgttttgcgattcctgccagctcccagg

SEQ ID NO: 423 - DNA, 40 bp, Homo sapiens
cccagtcattcaacaggaaggattcctgccagctcccagg

SEQ ID NO: 424 - DNA, 40 bp, Homo sapiens
gatgaatgctgacatggatgatctctctgcaagagtagat

SEQ ID NO: 425 - DNA, 40 bp, Homo sapiens
gatgaatgctgacatggatgcagttgatgctgaaaatcaa

SEQ ID NO: 426 - DNA, 40 bp, Homo sapiens
gtcaatgcttccatgtccagctttctgtcttctaggttcc

SEQ ID NO: 427 - DNA, 40 bp, Homo sapiens
gtcaatgcttccatgtccaggttccctccccatatggtcc

SEQ ID NO: 428 - DNA, 40 bp, Homo sapiens
tatggcaaggaggtcgaccttctctttcccagctgggcct

SEQ ID NO: 429 - DNA, 40 bp, Homo sapiens
tatggcaaggaggtcgacctctgggcctgtggggtgatct

SEQ ID NO: 430 - DNA, 40 bp, Homo sapiens
tggttttacctcggatagagacatttgttatcgctgtggt

SEQ ID NO: 431 - DNA, 40 bp, Homo sapiens
tggttttacctcggatagaggtttccagtttgtttcctcg

SEQ ID NO: 432 - DNA, 40 bp, Homo sapiens
gaatccgtatctgggaacagagccctttgctcctccctca

SEQ ID NO: 433 - DNA, 40 bp, Homo sapiens
gaatccgtatctgggaacagaatgaacggagaccagaatt

SEQ ID NO: 434 - DNA, 40 bp, Homo sapiens
tccaggagttccaggttccgtgtttcacttcaagcccact

SEQ ID NO: 435 - DNA, 40 bp, Homo sapiens
tttgactagggtccaaccagtgtttcacttcaagcccact

SEQ ID NO: 436 - DNA, 40 bp, Homo sapiens
gggcctgatgaatgacatcgcttcctcggcagtcatggga

SEQ ID NO: 437 - DNA, 40 bp, Homo sapiens
gggcctgatgaatgacatcgcagccttccctgcacccacc

SEQ ID NO: 438 - DNA, 40 bp, Homo sapiens
agccccaggatgcctcgcagctctcggaagaactggttgt

SEQ ID NO: 439 - DNA, 40 bp, Homo sapiens
agccccaggatgcctcgcagacgtgccttctgccatgatt

SEQ ID NO: 440 - DNA, 40 bp, Homo sapiens
acttgcctgtgaatttcgagtctttccctctgaaacaggt

SEQ ID NO: 441 - DNA, 40 bp, Homo sapiens
acttgcctgtgaatttcgaggtggcccgggagagtggccc

SEQ ID NO: 442 - DNA, 40 bp, Homo sapiens
tacccgggacaaccccaaggccgcccaccccaccccccat

SEQ ID NO: 443 - DNA, 40 bp, Homo sapiens
tacccgggacaaccccaaggggctctgtgacctctgcccc

SEQ ID NO: 444 - DNA, 40 bp, Homo sapiens
catagtggaagtgatagatcttctttttcacattacagtg

SEQ ID NO: 445 - DNA, 40 bp, Homo sapiens
catagtggaagtgatagatctggcctgaagcacgaggaca

SEQ ID NO: 446 - DNA, 40 bp, Homo sapiens
gctgtaccttcaggaacaggccctttctcccaggtttcca

SEQ ID NO: 447 - DNA, 40 bp, Homo sapiens
gctgtaccttcaggaacagggtttccatgctgagctcctg

SEQ ID NO: 448 - DNA, 40 bp, Homo sapiens
taaagcgactcattgagcaggaggtggtataacagacaga

SEQ ID NO: 449 - DNA, 40 bp, Homo sapiens
taaagcgactcattgagcaggcaaaaggcaggattgtggt

SEQ ID NO: 450 - DNA, 40 bp, Homo sapiens
tgggaatctggccagagaagtctttctgtcttgttttgaa

SEQ ID NO: 451 - DNA, 40 bp, Homo sapiens
tgggaatctggccagagaaggtgcttgacatcctccagca

SEQ ID NO: 452 - DNA, 40 bp, Homo sapiens
agaaaacatcgaattcagagcttgataatggaactataca

SEQ ID NO: 453 - DNA, 40 bp, Homo sapiens
agaaaacatcgaattcagagagttccagaagacagcgaac

SEQ ID NO: 454 - DNA, 40 bp, Homo sapiens
cgtccgccagtcgtcccgaggcatgaagaactcttgactg

SEQ ID NO: 455 - DNA, 40 bp, Homo sapiens
agccgggcgttgggggaaaggcatgaagaactcttgactg

SEQ ID NO: 456 - DNA, 40 bp, Homo sapiens
actaatcttcagcatgccattcggcgtggcacaagcctaa

SEQ ID NO: 457 - DNA, 40 bp, Homo sapiens
caaacacctcttgattataatcggcgtggcacaagcctaa

SEQ ID NO: 458 - DNA, 40 bp, Homo sapiens
caccacaaaatcacagacagcttgcttgccttttgtttta

SEQ ID NO: 459 - DNA, 40 bp, Homo sapiens
caccacaaaatcacagacagcagctgcagtatctcggaag

SEQ ID NO: 460 - DNA, 40 bp, Homo sapiens
ctcctactacacaatctaagatttcagaaatggccaaaga

SEQ ID NO: 461 - DNA, 40 bp, Homo sapiens
agagctcaaagaagtgtttaatttcagaaatggccaaaga

SEQ ID NO: 462 - DNA, 40 bp, Homo sapiens
atttccagaggatttacacttttgcttgacagggtcagtg

SEQ ID NO: 463 - DNA, 40 bp, Homo sapiens
atttccagaggatttacactggtcagtgctgcttgcccat

SEQ ID NO: 464 - DNA, 40 bp, Homo sapiens
gagtcggcgccgagaacatgtttcctgtgggccgcatcca

SEQ ID NO: 465 - DNA, 40 bp, Homo sapiens
cacagagagctgggctacagtttcctgtgggccgcatcca

SEQ ID NO: 466 - DNA, 40 bp, Homo sapiens
tgacgttctctgtgctccagtggtttctcccacaggttcc

SEQ ID NO: 467 - DNA, 40 bp, Homo sapiens
tgacgttctctgtgctccaggttcccggcccccaagtcgc

SEQ ID NO: 468 - DNA, 40 bp, Homo sapiens
caaacacctcttgattataacacgcaggtaacatggatgt

SEQ ID NO: 469 - DNA, 40 bp, Homo sapiens
tactccagcttcagcaacagcacctacagaagcggctcaa

SEQ ID NO: 470 - DNA, 40 bp, Homo sapiens
tactccagcttcagcaacagcaggtgataccctgtcggtc

SEQ ID NO: 471 - DNA, 40 bp, Homo sapiens
tctcagctgacgaatgcaaggcaccaacggagagacagct

SEQ ID NO: 472 - DNA, 40 bp, Homo sapiens
ggcatgcaaccaggcaccaggcaccaacggagagacagct

SEQ ID NO: 473 - DNA, 40 bp, Homo sapiens
tcaaatcatttacctccaagcagccagctcctgtcaccat

SEQ ID NO: 474 - DNA, 40 bp, Homo sapiens
tcaaatcatttacctccaagaggactcctgatggatttga

SEQ ID NO: 475 - DNA, 40 bp, Homo sapiens
agcaaaaaggggtgtctcagaatctccggcctgtgaaact

SEQ ID NO: 476 - DNA, 40 bp, Homo sapiens
agcaaaaaggggtgtctcaggccactcttcacctccacca

SEQ ID NO: 477 - DNA, 40 bp, Homo sapiens
tgttgcctccgcggccgcaggacagcaggtgccaggcttc

SEQ ID NO: 478 - DNA, 40 bp, Homo sapiens
tggtcatggccaaaccctgggacagcaggtgccaggcttc

SEQ ID NO: 479 - DNA, 40 bp, Homo sapiens
tgcctaaggcggatttgaatctctttctctcccttcagaa

SEQ ID NO: 480 - DNA, 40 bp, Homo sapiens
tgcctaaggcggatttgaataatcttatcttggctttgga

SEQ ID NO: 481 - DNA, 40 bp, Homo sapiens
tggtcatggccaaaccctgggctccaccctcatccagctg

SEQ ID NO: 482 - DNA, 40 bp, Homo sapiens
tgcagattccaaaagaaacgaaagcagaagatgaggatat

SEQ ID NO: 483 - DNA, 40 bp, Homo sapiens
ccttccacccaagggaactgaaagcagaagatgaggatat

SEQ ID NO: 484 - DNA, 40 bp, Homo sapiens
aggagggccccctgccgctggcaacaactcccagccctgc

SEQ ID NO: 485 - DNA, 40 bp, Homo sapiens
aggagggccccctgccgctgctgacccctttggcccgctt

SEQ ID NO: 486 - DNA, 40 bp, Homo sapiens
aacaactgcccagctttgagtggcaataatattgaactgg

SEQ ID NO: 487 - DNA, 40 bp, Homo sapiens
aacaactgcccagctttgaggaaatctgaaatagagtact

SEQ ID NO: 488 - DNA, 40 bp, Homo sapiens
gttgtgcccatgacctccaggttaggattaattgagtggc

SEQ ID NO: 489 - DNA, 40 bp, Homo sapiens
gttgtgcccatgacctccagtgatcccagggcaccgccgt

SEQ ID NO: 490 - DNA, 40 bp, Homo sapiens
gttaatgggtttaatggagagggcggcgaagaggacccgc

SEQ ID NO: 491 - DNA, 40 bp, Homo sapiens
gttaatgggtttaatggagatgagaaggcaaccaaagtgc

SEQ ID NO: 492 - DNA, 40 bp, Homo sapiens
gcaaggagcaacagcgatggtgagaaggcaaccaaagtgc

SEQ ID NO: 493 - DNA, 40 bp, Homo sapiens
agtttgagatgaagcgaatggatcctggcttcctggacaa

SEQ ID NO: 494 - DNA, 40 bp, Homo sapiens
agtttgagatgaagcgaatgctccccctaccaggggtcgc

SEQ ID NO: 495 - DNA, 40 bp, Homo sapiens
agaaaccttgaacgacaaagtggaatttttatactgtgac

SEQ ID NO: 496 - DNA, 40 bp, Homo sapiens
agaaaccttgaacgacaaagagacgtgagtcttgctgtgt

SEQ ID NO: 497 - DNA, 40 bp, Homo sapiens
acccctttggcatcgatcctgccctttcctcagcacaaga

SEQ ID NO: 498 - DNA, 40 bp, Homo sapiens
acccctttggcatcgatcctatttggagcctggctgccaa

SEQ ID NO: 499 - DNA, 40 bp, Homo sapiens
taaagtgttggctttacttaaatttatctttacagatact

SEQ ID NO: 500 - DNA, 40 bp, Homo sapiens
taaagtgttggctttacttaatactgcaaacaatttagtt

SEQ ID NO: 501 - DNA, 40 bp, Homo sapiens
acctcgtcagaaacaaccagagttcccccgtttctagagg

SEQ ID NO: 502 - DNA, 40 bp, Homo sapiens
acctcgtcagaaacaaccagaggttggaccagcctcaatg

SEQ ID NO: 503 - DNA, 40 bp, Homo sapiens
aaagatttcagaagaaatactatttctctttcaggtatac

SEQ ID NO: 504 - DNA, 40 bp, Homo sapiens
aaagatttcagaagaaatacgtataccaactgcagcctta

SEQ ID NO: 505 - DNA, 40 bp, Homo sapiens
ccaaaagaggggataatgagggaaggtgaagaaggagctg

SEQ ID NO: 506 - DNA, 40 bp, Homo sapiens
tcatcttgaaaaatgaaaattcctattttacagctgagga

SEQ ID NO: 507 - DNA, 40 bp, Homo sapiens
tcatcttgaaaaatgaaaatgtggataggcatgtagacct

SEQ ID NO: 508 - DNA, 40 bp, Homo sapiens
accctgtctaccagcctgtgttttctgccacctacaggat

SEQ ID NO: 509 - DNA, 40 bp, Homo sapiens
accctgtctaccagcctgtggatagaccatgaagctgaag

SEQ ID NO: 510 - DNA, 40 bp, Homo sapiens
tgacacagccctgcaggcagggtccgtgcaggacctttcc

SEQ ID NO: 511 - DNA, 40 bp, Homo sapiens
tgacacagccctgcaggcagaaggatcccgcaaacgtgga

SEQ ID NO: 512 - DNA, 40 bp, Homo sapiens
gcggggcgagggcagctccgcgtttctctgaattctcccc

SEQ ID NO: 513 - DNA, 40 bp, Homo sapiens
gcggggcgagggcagctccgggaaggaacgtcccagggat

SEQ ID NO: 514 - DNA, 40 bp, Homo sapiens
ccacctcaccatcacccagggcagcccctccacagggccc

SEQ ID NO: 515 - DNA, 40 bp, Homo sapiens
ccacctcaccatcacccaggccctcaggcagcccctccac

SEQ ID NO: 516 - DNA, 40 bp, Homo sapiens
gccaacctagagcccccctgctctctgcctcttacagatg

SEQ ID NO: 517 - DNA, 40 bp, Homo sapiens
gccaacctagagcccccctgatgactggcatagcctgggc

SEQ ID NO: 518 - DNA, 40 bp, Homo sapiens
aaccgggggagcgaggcacgtttctttccccacctttcta

SEQ ID NO: 519 - DNA, 40 bp, Homo sapiens
aaccgggggagcgaggcacggagtgtacctcacagccttc

SEQ ID NO: 520 - DNA, 40 bp, Homo sapiens
cacacagactgcgttcgatgagtgtcttccccctgcctta

SEQ ID NO: 521 - DNA, 40 bp, Homo sapiens
cacacagactgcgttcgatgccttgctgttcaccctgatg

SEQ ID NO: 522 - DNA, 40 bp, Homo sapiens
gtttttacctctgcctcctgatctctcatcctaggttttc

SEQ ID NO: 523 - DNA, 40 bp, Homo sapiens
gtttttacctctgcctcctggttttcatactctgcacacc

SEQ ID NO: 524 - DNA, 40 bp, Homo sapiens
cactgctgggagagtggaagttgcttccacagattcctga

SEQ ID NO: 525 - DNA, 40 bp, Homo sapiens
cactgctgggagagtggaagattcctgagagctgccggcc

SEQ ID NO: 526 - DNA, 40 bp, Homo sapiens
gattttggagaggcaaccaactttgtttttcacagattcc

SEQ ID NO: 527 - DNA, 40 bp, Homo sapiens
gattttggagaggcaaccaaattccctggactttgtcacc

SEQ ID NO: 528 - DNA, 40 bp, Homo sapiens
tgcagaactggataaagaagtgtatttttttgtctcaatt

SEQ ID NO: 529 - DNA, 40 bp, Homo sapiens
tgcagaactggataaagaaggtgcttctaaagtaaagaaa

SEQ ID NO: 530 - DNA, 40 bp, Homo sapiens
actcttatgcagtccccatgaggttatgcttatgtttctc

SEQ ID NO: 531 - DNA, 40 bp, Homo sapiens
actcttatgcagtccccatgaggagatcctagtctcacca

SEQ ID NO: 532 - DNA, 40 bp, Homo sapiens
agtgttttaccatggatgttgtcattccagggctcctcag

SEQ ID NO: 533 - DNA, 40 bp, Homo sapiens
agtgttttaccatggatgttggctcctcagtggctgtgac

SEQ ID NO: 534 - DNA, 40 bp, Homo sapiens
tttatgatgctgctttaaagttttgttaatgtttttcttt

SEQ ID NO: 535 - DNA, 40 bp, Homo sapiens
tttatgatgctgctttaaagctcattaatgaaattgaaga

SEQ ID NO: 536 - DNA, 40 bp, Homo sapiens
atctaaaaacagaagagcaggtccttttttaggtgcaaaa

SEQ ID NO: 537 - DNA, 40 bp, Homo sapiens
atctaaaaacagaagagcaggtgcaaaaacttcaagctat

SEQ ID NO: 538 - DNA, 40 bp, Homo sapiens
ggattgcagccaacacaaagtttctcttcataggaatgtc

SEQ ID NO: 539 - DNA, 40 bp, Homo sapiens
ggattgcagccaacacaaaggaatgtcccaaatgccatgt

SEQ ID NO: 540 - DNA, 40 bp, Homo sapiens
ggtttcgagtttgaatagtgttttgcttgtttgtttgttt

SEQ ID NO: 541 - DNA, 40 bp, Homo sapiens
ggtttcgagtttgaatagtggtcagattgaagttatcatg

SEQ ID NO: 542 - DNA, 40 bp, Homo sapiens
cgcaagtacttcctgccccatccagcagcacacagtggga

SEQ ID NO: 543 - DNA, 40 bp, Homo sapiens
cgcaagtacttcctgccccaggtagtggtgactgtgaacc

SEQ ID NO: 544 - DNA, 40 bp, Homo sapiens
ttcataacaaaccagtaaatcacattcaggaattcaccaa

SEQ ID NO: 545 - DNA, 40 bp, Homo sapiens
tcatcaatgccccgaccttgcacattcaggaattcaccaa

SEQ ID NO: 546 - DNA, 40 bp, Homo sapiens
aaatttaacattactcatagtttttgctgttttacagagt

SEQ ID NO: 547 - DNA, 40 bp, Homo sapiens
aaatttaacattactcatagagtaagccatatcaaagact

SEQ ID NO: 548 - DNA, 40 bp, Homo sapiens
caccgggagctgcagggccgccccttgtccatcccaggca

SEQ ID NO: 549 - DNA, 40 bp, Homo sapiens
caccgggagctgcagggccggcacgagcagctgcaggccc

SEQ ID NO: 550 - DNA, 40 bp, Homo sapiens
attggacacagagatgggatatcgtgacgtctgcatccac

SEQ ID NO: 551 - DNA, 40 bp, Homo sapiens
ctgtctctaggctaagcagaatcgtgacgtctgcatccac

SEQ ID NO: 552 - DNA, 40 bp, Homo sapiens
gggacctcaccaagcgcccgcccctcatcaacctgcagat

SEQ ID NO: 553 - DNA, 40 bp, Homo sapiens
gggacctcaccaagcgcccgatctgcaggcaggccctgaa

SEQ ID NO: 554 - DNA, 40 bp, Homo sapiens
gagtgtgaatcatctgtgaatttcacatcactcatttaac

SEQ ID NO: 555 - DNA, 40 bp, Homo sapiens
gagtgtgaatcatctgtgaaccagctgaaagaaacattgg

SEQ ID NO: 556 - DNA, 40 bp, Homo sapiens
tcatcaatgccccgaccttggttcatgaacacattgaggt

SEQ ID NO: 557 - DNA, 40 bp, Homo sapiens
gcatttctgagaaggctcgggtcctctcccgcaggggctg

SEQ ID NO: 558 - DNA, 40 bp, Homo sapiens
gcatttctgagaaggctcgggggctggctttgacctacag

SEQ ID NO: 559 - DNA, 40 bp, Homo sapiens
gccagtccagagccctcaagttcttcttctcagctcttgt

SEQ ID NO: 560 - DNA, 40 bp, Homo sapiens
gccagtccagagccctcaagctcttgtggccatggagaag

SEQ ID NO: 561 - DNA, 40 bp, Homo sapiens
tggccgaggcgctgaccaagaccttactcaggggatcctc

SEQ ID NO: 562 - DNA, 40 bp, Homo sapiens
tggccgaggcgctgaccaaggctgagggcagaggaggcct

SEQ ID NO: 563 - DNA, 40 bp, Homo sapiens
tctacttggtgggcttcttgcatttattttgttttaggat

SEQ ID NO: 564 - DNA, 40 bp, Homo sapiens
tctacttggtgggcttcttggatttgtttggtgtcagcat

SEQ ID NO: 565 - DNA, 40 bp, Homo sapiens
gctcctgctcagtatatccgtttttatctgctttcttcag

SEQ ID NO: 566 - DNA, 40 bp, Homo sapiens
gctcctgctcagtatatccgatacacaccatctcagcaag

SEQ ID NO: 567 - DNA, 40 bp, Homo sapiens
gaaatagggcacagatccagtttttctttaattttagact

SEQ ID NO: 568 - DNA, 40 bp, Homo sapiens
gaaatagggcacagatccagactgtgatagatgccaacat

SEQ ID NO: 569 - DNA, 40 bp, Homo sapiens
gcaacctgtgttttacaaaggttttattttttagatggtg

SEQ ID NO: 570 - DNA, 40 bp, Homo sapiens
gcaacctgtgttttacaaagatggtgtcctacagcagcca

SEQ ID NO: 571 - DNA, 40 bp, Homo sapiens
cccctgaagtactagcaaagcatgttaatattttataggt

SEQ ID NO: 572 - DNA, 40 bp, Homo sapiens
cccctgaagtactagcaaaggtacaggcaattaaacttct

SEQ ID NO: 573 - DNA, 40 bp, Homo sapiens
gttcctcactttgaatgaggtgtttttgattctgcaggtg

SEQ ID NO: 574 - DNA, 40 bp, Homo sapiens
gttcctcactttgaatgagggtgcatggtactcagtaggt

SEQ ID NO: 575 - DNA, 40 bp, Homo sapiens
tcttggaaggcagagaaaagatatttctagagcatttggg

SEQ ID NO: 576 - DNA, 40 bp, Homo sapiens
tcttggaaggcagagaaaagtctacctcgagacctatggc

SEQ ID NO: 577 - DNA, 40 bp, Homo sapiens
aacccggagagaaaagggagtttgtttttaggtcagagtc

SEQ ID NO: 578 - DNA, 40 bp, Homo sapiens
aacccggagagaaaagggagcaactgatgttgccatgcag

SEQ ID NO: 579 - DNA, 40 bp, Homo sapiens
aatcttccccaagatgtatgttctatgttccagcagagat

SEQ ID NO: 580 - DNA, 40 bp, Homo sapiens
aatcttccccaagatgtatggttatatcaatcagtgaaaa

SEQ ID NO: 581 - DNA, 40 bp, Homo sapiens
ctctcttgtcagacaagcagttgtctcttccaggtaatgg

SEQ ID NO: 582 - DNA, 40 bp, Homo sapiens
ctctcttgtcagacaagcaggtaatggagactatacagtg

SEQ ID NO: 583 - DNA, 40 bp, Homo sapiens
gcagagctgtggcttaccagtccctccttgttccagatgt

SEQ ID NO: 584 - DNA, 40 bp, Homo sapiens
gcagagctgtggcttaccagatgtggcaaaatctggcaaa

SEQ ID NO: 585 - DNA, 40 bp, Homo sapiens
tgcaggagaccggcttttgggtccccttcttatacccctc

SEQ ID NO: 586 - DNA, 40 bp, Homo sapiens
tgcaggagaccggcttttggatactgctaatcagtcctag

SEQ ID NO: 587 - DNA, 40 bp, Homo sapiens
tcttgccagagctgcccacgctctccaccctcagctgcct

SEQ ID NO: 588 - DNA, 40 bp, Homo sapiens
tcttgccagagctgcccacgcttctttccttgctgctgga

SEQ ID NO: 589 - DNA, 40 bp, Homo sapiens
gcaggctgcccgggactctggctctctttctctcagggga

SEQ ID NO: 590 - DNA, 40 bp, Homo sapiens
gcaggctgcccgggactctggggacatgaagggacagtgg

SEQ ID NO: 591 - DNA, 40 bp, Homo sapiens
gccagtccagagccctcaagtctttaccagacttgcaggg

SEQ ID NO: 592 - DNA, 40 bp, Homo sapiens
ttcccactggtcgcctgcaggtatttctctttagactggc

SEQ ID NO: 593 - DNA, 40 bp, Homo sapiens
ttcccactggtcgcctgcagactggcatccttcgaaccaa

SEQ ID NO: 594 - DNA, 40 bp, Homo sapiens
tgtaaatggggaagcgctgttttctacagactgccattgc

SEQ ID NO: 595 - DNA, 40 bp, Homo sapiens
tgtaaatggggaagcgctgtgcgacgactgtaagggcaag

SEQ ID NO: 596 - DNA, 40 bp, Homo sapiens
tcaatgcaaatatcatcatggattttcttcctaaatttct

SEQ ID NO: 597 - DNA, 40 bp, Homo sapiens
tcaatgcaaatatcatcatgcctgaatttgaaaccaagtg

SEQ ID NO: 598 - DNA, 40 bp, Homo sapiens
acaaatcaactggaaagcaattactgttttcaggcagtct

SEQ ID NO: 599 - DNA, 40 bp, Homo sapiens
acaaatcaactggaaagcaagcagtctgcagaactaaata

SEQ ID NO: 600 - DNA, 40 bp, Homo sapiens
caaagcgcccagccctgggggctggaggctgagccccggc

SEQ ID NO: 601 - DNA, 40 bp, Homo sapiens
caaagcgcccagccctggggatccggaaacggcactcaag

SEQ ID NO: 602 - DNA, 40 bp, Homo sapiens
tgacacagccctgcaggcaggacctttccccctccctagt

SEQ ID NO: 603 - DNA, 40 bp, Homo sapiens
agttgccattccattacatgtctttactttcctgaagctt

SEQ ID NO: 604 - DNA, 40 bp, Homo sapiens
agttgccattccattacatgcttcaagcttagatgatgtt

SEQ ID NO: 605 - DNA, 40 bp, Homo sapiens
actgattaaaaatcttggtggtgatttctctttgccagtt

SEQ ID NO: 606 - DNA, 40 bp, Homo sapiens
actgattaaaaatcttggtgttgatacaatacaaatggaa

SEQ ID NO: 607 - DNA, 40 bp, Homo sapiens
aggctattgttgcagaccgggctgttttccttacagatgg

SEQ ID NO: 608 - DNA, 40 bp, Homo sapiens
aggctattgttgcagaccggatggtagaaatcctattcca

SEQ ID NO: 609 - DNA, 40 bp, Homo sapiens
cctttcaagaaaacaaaaagtcgctttttccagtggcggt

SEQ ID NO: 610 - DNA, 40 bp, Homo sapiens
cctttcaagaaaacaaaaaggcaaagtgctcttaggagaa

SEQ ID NO: 611 - DNA, 40 bp, Homo sapiens
acacggagctcaagaaacagtttcttccagaactaccagc

SEQ ID NO: 612 - DNA, 40 bp, Homo sapiens
acacggagctcaagaaacagatggcaaaccaaaaagattt

SEQ ID NO: 613 - DNA, 40 bp, Homo sapiens
gacttcgaacatttaaacagtgtgttacaggtagaagaga

SEQ ID NO: 614 - DNA, 40 bp, Homo sapiens
gacttcgaacatttaaacagaggtatcctgggcaagtcat

SEQ ID NO: 615 - DNA, 40 bp, Homo sapiens
accacgaagggtcacacaagtctatttggtccaggggcag

SEQ ID NO: 616 - DNA, 40 bp, Homo sapiens
accacgaagggtcacacaaggggcagcctcacctgggcat

SEQ ID NO: 617 - DNA, 40 bp, Homo sapiens
ttaacaaacacgtgaatctacagtgtttggccagcgcttg

SEQ ID NO: 618 - DNA, 40 bp, Homo sapiens
tgctggcacaccctgtggagcagtgtttggccagcgcttg

SEQ ID NO: 619 - DNA, 40 bp, Homo sapiens
cgccccagggcaagcgaaaggtgttccttgacttgtgcgt

SEQ ID NO: 620 - DNA, 40 bp, Homo sapiens
cgccccagggcaagcgaaaggtgatcaacactccggaaat

SEQ ID NO: 621 - DNA, 40 bp, Homo sapiens
tggtacaacttcaggaaaagtctgtttgttttgcagtgtt

SEQ ID NO: 622 - DNA, 40 bp, Homo sapiens
tggtacaacttcaggaaaagtgtttagccctccaggccca

SEQ ID NO: 623 - DNA, 40 bp, Homo sapiens
tggatttgctcggcttttgattttgattccagccttccgc

SEQ ID NO: 624 - DNA, 40 bp, Homo sapiens
tggatttgctcggcttttgactggaccgagtgactactat

SEQ ID NO: 625 - DNA, 40 bp, Homo sapiens
gatgaggacccccacataggtttccaaaccaggatggcca

SEQ ID NO: 626 - DNA, 40 bp, Homo sapiens
gatgaggacccccacatagggatggccatagcagccacaa

SEQ ID NO: 627 - DNA, 40 bp, Homo sapiens
tgttttaaattccatagcagctatttctacagtaaaccat

SEQ ID NO: 628 - DNA, 40 bp, Homo sapiens
tgttttaaattccatagcagcattttcatcaatagctatt

SEQ ID NO: 629 - DNA, 40 bp, Homo sapiens
gctgggatgttagggctcagcctgtcgttccaggacccag

SEQ ID NO: 630 - DNA, 40 bp, Homo sapiens
gctgggatgttagggctcagggaagaaaagtcagaagacc

SEQ ID NO: 631 - DNA, 40 bp, Homo sapiens
ctggttattgcaaattaaagctctttgccgtcccctccta

SEQ ID NO: 632 - DNA, 40 bp, Homo sapiens
ctggttattgcaaattaaaggtcttcaaccccaggattgg

SEQ ID NO: 633 - DNA, 40 bp, Homo sapiens
ggtcatgctaatgagacaggtctgttgtttttttagattt

SEQ ID NO: 634 - DNA, 40 bp, Homo sapiens
ggtcatgctaatgagacaggatttgatgaggcgccaagaa

SEQ ID NO: 635 - DNA, 40 bp, Homo sapiens
gtcagcatttgcagactttgtttcttttggcagatggaga

SEQ ID NO: 636 - DNA, 40 bp, Homo sapiens
gtcagcatttgcagactttgatggagatggacacatggat

SEQ ID NO: 637 - DNA, 40 bp, Homo sapiens
gcagagctgtggcttaccagacttctccctttccaggccc

SEQ ID NO: 638 - DNA, 40 bp, Homo sapiens
tgcagctggcccccgcccaggtcttttctctcccacaggc

SEQ ID NO: 639 - DNA, 40 bp, Homo sapiens
tgcagctggcccccgcccaggcccctgtctcccagcctga

SEQ ID NO: 640 - DNA, 40 bp, Homo sapiens
cacagcaagcaccttctgagttcttttcttatttcaggct

SEQ ID NO: 641 - DNA, 40 bp, Homo sapiens
cacagcaagcaccttctgaggctgatttggagcaatataa

SEQ ID NO: 642 - DNA, 40 bp, Homo sapiens
tcacacctgtaggaactgagtgtattatgatacaggaaga

SEQ ID NO: 643 - DNA, 40 bp, Homo sapiens
tcacacctgtaggaactgaggaagaagttatggcagaaga

SEQ ID NO: 644 - DNA, 40 bp, Homo sapiens
aaaattgactatggcaacaatttttgctttacagaatcct

SEQ ID NO: 645 - DNA, 40 bp, Homo sapiens
aaaattgactatggcaacaaaatccttgagcttgatttga

SEQ ID NO: 646 - DNA, 40 bp, Homo sapiens
acacggagctcaagaaacagaactaccagcagatctagaa

SEQ ID NO: 647 - DNA, 40 bp, Homo sapiens
gggaggaaaagtaattaatgtttttgtttttcttttttag

SEQ ID NO: 648 - DNA, 40 bp, Homo sapiens
gggaggaaaagtaattaatggaagttatagaactaaccaa

SEQ ID NO: 649 - DNA, 40 bp, Homo sapiens
agaaggagctgcagggccagtgtttccttcacagaatgtg

SEQ ID NO: 650 - DNA, 40 bp, Homo sapiens
agaaggagctgcagggccagaatgtggaggctgtggaccc

SEQ ID NO: 651 - DNA, 40 bp, Homo sapiens
gctctggagaatctcaataaggtttttcttcctttagggc

SEQ ID NO: 652 - DNA, 40 bp, Homo sapiens
gctctggagaatctcaataaggctctcctagcagacattg

SEQ ID NO: 653 - DNA, 40 bp, Homo sapiens
catgcaatgaacccaaaaggttgattccagtgctaaaagg

SEQ ID NO: 654 - DNA, 40 bp, Homo sapiens
catgcaatgaacccaaaaggtcactctgagaggagtgata

SEQ ID NO: 655 - DNA, 40 bp, Homo sapiens
tgcttccggaacagtgacagccccatctctgcccctgcta

SEQ ID NO: 656 - DNA, 40 bp, Homo sapiens
tgcttccggaacagtgacagggacttcgcttttgtggcaa

SEQ ID NO: 657 - DNA, 40 bp, Homo sapiens
tgggtttcagcaagagaacattgtttttctgattttctag

SEQ ID NO: 658 - DNA, 40 bp, Homo sapiens
tgggtttcagcaagagaacactggcagcctcaggaaacaa

SEQ ID NO: 659 - DNA, 40 bp, Homo sapiens
aggacatggatttggtagagtgctctaatttttgttttaa

SEQ ID NO: 660 - DNA, 40 bp, Homo sapiens
aggacatggatttggtagaggtgaatgaagcttttgctcc

SEQ ID NO: 661 - DNA, 40 bp, Homo sapiens
atcacaaccggaaccgcaggctccttctgccctgcccgca

SEQ ID NO: 662 - DNA, 40 bp, Homo sapiens
atcacaaccggaaccgcaggctcatgatggagcagtccaa

SEQ ID NO: 663 - DNA, 40 bp, Homo sapiens
caggaagcagctagtcttttatgtttattctctttgtaga

SEQ ID NO: 664 - DNA, 40 bp, Homo sapiens
caggaagcagctagtcttttaggtaagaagtatggagaga

SEQ ID NO: 665 - DNA, 40 bp, Homo sapiens
gaaccaatggaatggagaaggcacaggcgttttgcaaagg

SEQ ID NO: 666 - DNA, 40 bp, Homo sapiens
gaaccaatggaatggagaaggtcctatggccgggctccga

SEQ ID NO: 667 - DNA, 40 bp, Homo sapiens
tgcttgtaaaattgaaatggtgcttttaattattatagtt

SEQ ID NO: 668 - DNA, 40 bp, Homo sapiens
tgcttgtaaaattgaaatggttgactacaaagaagaatat

SEQ ID NO: 669 - DNA, 40 bp, Homo sapiens
ccacctcaccatcacccaggcccctccacagggcccctct

SEQ ID NO: 670 - DNA, 40 bp, Homo sapiens
cgtctccatgaccatgcaaggtgtagacgcagtgctcccc

SEQ ID NO: 671 - DNA, 40 bp, Homo sapiens
cgtctccatgaccatgcaaggcttcctgaactactacgat

SEQ ID NO: 672 - DNA, 40 bp, Homo sapiens
aggaggcaattaaggcaaaggccctttccctgctacaggt

SEQ ID NO: 673 - DNA, 40 bp, Homo sapiens
aggaggcaattaaggcaaaggtggggcagtacgtgtcccg

SEQ ID NO: 674 - DNA, 40 bp, Homo sapiens
ttacctccgaaggatcgtggttctctttgtagggtctgcc

SEQ ID NO: 675 - DNA, 40 bp, Homo sapiens
ttacctccgaaggatcgtggggtctgccacaaggtacctc

SEQ ID NO: 676 - DNA, 40 bp, Homo sapiens
aataagccctcagatggcagcctgtctgacctgtgggccc

SEQ ID NO: 677 - DNA, 40 bp, Homo sapiens
aataagccctcagatggcaggcccaagtatctggtggtga

SEQ ID NO: 678 - DNA, 40 bp, Homo sapiens
gcctggacctgtacttggaggtgcagatccaggcgtacct

SEQ ID NO: 679 - DNA, 40 bp, Homo sapiens
gcctggacctgtacttggagaggcttcggctcaccgagag

SEQ ID NO: 680 - DNA, 40 bp, Homo sapiens
ctgtaactactagcccacagtttcttttttattcaaatag

SEQ ID NO: 681 - DNA, 40 bp, Homo sapiens
ctgtaactactagcccacagagtgacatgatgagggagca

SEQ ID NO: 682 - DNA, 40 bp, Homo sapiens
ctctcaatgcagctttacagttttcctgcagattgttcaa

SEQ ID NO: 683 - DNA, 40 bp, Homo sapiens
ctctcaatgcagctttacaggcttcaatggctgagaatag

SEQ ID NO: 684 - DNA, 40 bp, Homo sapiens
ggagcagttccagaagactgctgcttctccatagggacca

SEQ ID NO: 685 - DNA, 40 bp, Homo sapiens
ggagcagttccagaagactgggaccattgttgtggaaggc

SEQ ID NO: 686 - DNA, 40 bp, Homo sapiens
cctgctggaccattcttacgttgtctccccctgttcctaa

SEQ ID NO: 687 - DNA, 40 bp, Homo sapiens
cctgctggaccattcttacgatttcaaccagctggatggt

SEQ ID NO: 688 - DNA, 40 bp, Homo sapiens
ggattttgataatgaagaagttgtgctctttttccagagg

SEQ ID NO: 689 - DNA, 40 bp, Homo sapiens
ggattttgataatgaagaagaggaacagtcagtccctccc

SEQ ID NO: 690 - DNA, 40 bp, Homo sapiens
cgtctccatgaccatgcaagggcaggtgtagacgcagtgc

SEQ ID NO: 691 - DNA, 40 bp, Homo sapiens
agtgccagctgcgggcccggctctcaccagtgacgccctc

SEQ ID NO: 692 - DNA, 40 bp, Homo sapiens
agtgccagctgcgggcccgggaatcgtacaagtacttccc

SEQ ID NO: 693 - DNA, 40 bp, Homo sapiens
aacttactttgtttatgatgcttttattttagattcagag

SEQ ID NO: 694 - DNA, 40 bp, Homo sapiens
aacttactttgtttatgatgagtatgaagatggtgatctg

SEQ ID NO: 695 - DNA, 40 bp, Homo sapiens
atcatagcccacatgtccagtttttctttctaggtaaaag

SEQ ID NO: 696 - DNA, 40 bp, Homo sapiens
atcatagcccacatgtccaggtaaaagcagcgtttaatga

SEQ ID NO: 697 - DNA, 40 bp, Homo sapiens
tgactccgctgctcgccatgactttcaggattaagcgatt

SEQ ID NO: 698 - DNA, 40 bp, Homo sapiens
tgactccgctgctcgccatgtcttctcacaagactttcag

SEQ ID NO: 699 - DNA, 40 bp, Homo sapiens
ccaagcacctgaaacagcagtttgcaggcttctattttag

SEQ ID NO: 700 - DNA, 40 bp, Homo sapiens
ccaagcacctgaaacagcagatgctgaaaaagttcacttc

SEQ ID NO: 701 - DNA, 40 bp, Homo sapiens
cgagctgttggcatccttggtttcttgtccacaggagaag

SEQ ID NO: 702 - DNA, 40 bp, Homo sapiens
cgagctgttggcatccttgggacctgccgctgccaagcca

SEQ ID NO: 703 - DNA, 40 bp, Homo sapiens
gctttctacggaacatcaatgagcttctgtctgcacacag

SEQ ID NO: 704 - DNA, 40 bp, Homo sapiens
gctttctacggaacatcaatgagtacctggccgtagtcga

SEQ ID NO: 705 - DNA, 40 bp, Homo sapiens
caggaatacctgcagataagatttcacagaatattcgcta

SEQ ID NO: 706 - DNA, 40 bp, Homo sapiens
caggaatacctgcagataagatgatagttactgatatata

SEQ ID NO: 707 - DNA, 40 bp, Homo sapiens
ctacaccaagaagagaggacctcttccctcgcgcagaatc

SEQ ID NO: 708 - DNA, 40 bp, Homo sapiens
ctacaccaagaagagaggacagaggccagacttcacagac

SEQ ID NO: 709 - DNA, 40 bp, Homo sapiens
cggaggctgtctcctctcagacttcctctctcccaccagg

SEQ ID NO: 710 - DNA, 40 bp, Homo sapiens
cggaggctgtctcctctcaggaaatgctgcgctgcatttg

SEQ ID NO: 711 - DNA, 40 bp, Homo sapiens
tcctgctggagccacccaagctttttcttcttcagaaaag

SEQ ID NO: 712 - DNA, 40 bp, Homo sapiens
tcctgctggagccacccaagaaaagtgtgatgaagaccac

SEQ ID NO: 713 - DNA, 40 bp, Homo sapiens
accaagcatacttccagatgttctctctatttaagggtca

SEQ ID NO: 714 - DNA, 40 bp, Homo sapiens
accaagcatacttccagatgggtcaatattctctcgagtt

SEQ ID NO: 715 - DNA, 40 bp, Homo sapiens
cgggccgcccccctgcccggtgttcttctgggcagtgcaa

SEQ ID NO: 716 - DNA, 40 bp, Homo sapiens
cgggccgcccccctgcccggaggccggtccctgccaaggg

SEQ ID NO: 717 - DNA, 40 bp, Homo sapiens
ggaggactggggtctgcagacatttcttgcagacagcacc

SEQ ID NO: 718 - DNA, 40 bp, Homo sapiens
ggaggactggggtctgcagaacagcaccttgtattctggc

SEQ ID NO: 719 - DNA, 40 bp, Homo sapiens
ctgccccctgcgccacacggcctctttccctgcagtgatg

SEQ ID NO: 720 - DNA, 40 bp, Homo sapiens
ctgccccctgcgccacacggtgatggttcattcgcatatg

SEQ ID NO: 721 - DNA, 40 bp, Homo sapiens
tgtaaatggggaagcgctgtactgccattgctatgcacgg

SEQ ID NO: 722 - DNA, 40 bp, Homo sapiens
ctgatgaaaactactacaagcagacaccttacaggccagg

SEQ ID NO: 723 - DNA, 40 bp, Homo sapiens
ctgatgaaaactactacaaggcccagacccatggaaagtg

SEQ ID NO: 724 - DNA, 40 bp, Homo sapiens
ttcagctgcccctgaagaagaaacatgttctccttccttc

SEQ ID NO: 725 - DNA, 40 bp, Homo sapiens
ttcagctgcccctgaagaaggaatgagtagcgacagtgac

SEQ ID NO: 726 - DNA, 40 bp, Homo sapiens
tcccgaagccacctcatgagcctctgccttcccccaggtc

SEQ ID NO: 727 - DNA, 40 bp, Homo sapiens
tcccgaagccacctcatgaggtcgggcagtgtgatggagc

SEQ ID NO: 728 - DNA, 40 bp, Homo sapiens
ccccggtgcgtaaggaggagcctgcccccctttggccctg

SEQ ID NO: 729 - DNA, 40 bp, Homo sapiens
ccccggtgcgtaaggaggaggaggacaatcccaaggggga

SEQ ID NO: 730 - DNA, 40 bp, Homo sapiens
agctggagaaaaaccttctttttcttccagaactaccagc

SEQ ID NO: 731 - DNA, 40 bp, Homo sapiens
agctggagaaaaaccttcttatggcaaaccaaaaagattt

SEQ ID NO: 732 - DNA, 40 bp, Homo sapiens
ttcgttggcagcttctgctgagaccctgacccccaccccc

SEQ ID NO: 733 - DNA, 40 bp, Homo sapiens
ttcgttggcagcttctgctgcgtccacagagaccctgacc

SEQ ID NO: 734 - DNA, 40 bp, Homo sapiens
gtgccaacgaggaccaggagttctttatttcagatggaac

SEQ ID NO: 735 - DNA, 40 bp, Homo sapiens
gtgccaacgaggaccaggagatggaactagaagcattacg

SEQ ID NO: 736 - DNA, 40 bp, Homo sapiens
cctcacgatgcaaggccacgagttcatgtcccacagggag

SEQ ID NO: 737 - DNA, 40 bp, Homo sapiens
cctcacgatgcaaggccacgggagaagctgtgtacactgt

SEQ ID NO: 738 - DNA, 40 bp, Homo sapiens
aaaaataaagcctttcccaggcccagacccatggaaagtg

SEQ ID NO: 739 - DNA, 40 bp, Homo sapiens
cgaggatgaagacagagcaggtgaccaagaaaaaaaagaa

SEQ ID NO: 740 - DNA, 40 bp, Homo sapiens
cgaggatgaagacagagcagtacaggtgaccaagaaaaaa

SEQ ID NO: 741 - DNA, 40 bp, Homo sapiens
aaaatgggctcagcagttagggttttttgttgtttgtttg

SEQ ID NO: 742 - DNA, 40 bp, Homo sapiens
aaaatgggctcagcagttagaccttttcacagatgctgct

SEQ ID NO: 743 - DNA, 40 bp, Homo sapiens
aagcactggcccagtgtcaggagccagattctgtgcgaga

SEQ ID NO: 744 - DNA, 40 bp, Homo sapiens
aagcactggcccagtgtcagaaggagccagattctgtgcg

SEQ ID NO: 745 - DNA, 40 bp, Homo sapiens
ccactctcacaatgacccaggaggacccccggcggcgctt

SEQ ID NO: 746 - DNA, 40 bp, Homo sapiens
ccactctcacaatgacccaggctggatcaagacctttgac

SEQ ID NO: 747 - DNA, 40 bp, Homo sapiens
cctttacttggggctctcagcaactgatgttgccatgcag

SEQ ID NO: 748 - DNA, 40 bp, Homo sapiens
actcagatgccgaaaactcgccctcagtctgaggttctgt

SEQ ID NO: 749 - DNA, 40 bp, Homo sapiens
actcagatgccgaaaactcgtgcatggagcccatggagac

SEQ ID NO: 750 - DNA, 40 bp, Homo sapiens
gcctactcttaaccattagggtggataggcatgtagacct

SEQ ID NO: 751 - DNA, 40 bp, Homo sapiens
tggagtgcggatttgcaacacttgcttccttctcccacat

SEQ ID NO: 752 - DNA, 40 bp, Homo sapiens
tggagtgcggatttgcaacaatcaaagatctgcgagacca

SEQ ID NO: 753 - DNA, 40 bp, Homo sapiens
caactggagttcattttcaggttttttgacagactatgta

SEQ ID NO: 754 - DNA, 40 bp, Homo sapiens
caactggagttcattttcagactatgtatgagcacttggg

SEQ ID NO: 755 - DNA, 40 bp, Homo sapiens
caatgtgttgaccatcgcagtccccctacagccctgttca

SEQ ID NO: 756 - DNA, 40 bp, Homo sapiens
caatgtgttgaccatcgcagcctctcctgccaacttacag

SEQ ID NO: 757 - DNA, 40 bp, Homo sapiens
cagctgctctcaggagagagtggactggctctgtaggtac

SEQ ID NO: 758 - DNA, 40 bp, Homo sapiens
cagctgctctcaggagagaggtacaaagaagacccctggc

SEQ ID NO: 759 - DNA, 40 bp, Homo sapiens
tctctagtgggcccttctagttctacaaggtaaaactcta

SEQ ID NO: 760 - DNA, 40 bp, Homo sapiens
tctctagtgggcccttctaggaatgaccaaaagaagacaa

SEQ ID NO: 761 - DNA, 40 bp, Homo sapiens
agctccgagagggcaaggagctccctccctcctagaaatg

SEQ ID NO: 762 - DNA, 40 bp, Homo sapiens
agctccgagagggcaaggagaaatgtgtccactactggcc

SEQ ID NO: 763 - DNA, 40 bp, Homo sapiens
gacgtggcagctcatgtgagcattgtgtcgttacaggctt

SEQ ID NO: 764 - DNA, 40 bp, Homo sapiens
gacgtggcagctcatgtgaggcttcagtgtcatttgagga

SEQ ID NO: 765 - DNA, 40 bp, Homo sapiens
aaggaagaacaagactttgtttagtgtgactctggatcca

SEQ ID NO: 766 - DNA, 40 bp, Homo sapiens
aatgttaaggagtcatcaagttagtgtgactctggatcca

SEQ ID NO: 767 - DNA, 40 bp, Homo sapiens
aggagaacaccttatttcagcttttatttttatgtgataa

SEQ ID NO: 768 - DNA, 40 bp, Homo sapiens
aggagaacaccttatttcagaaaaggtgtaccatacctga

SEQ ID NO: 769 - DNA, 40 bp, Homo sapiens
ctgatgaaaactactacaagacaccttacaggccaggaga

SEQ ID NO: 770 - DNA, 40 bp, Homo sapiens
ggggccaccaggttggccagcggccccctttcccagggcc

SEQ ID NO: 771 - DNA, 40 bp, Homo sapiens
ggggccaccaggttggccagggccatggctgagcacgcag

SEQ ID NO: 772 - DNA, 40 bp, Homo sapiens
tgcacacgcctctcctacagagtctcttatgctggtccca

SEQ ID NO: 773 - DNA, 40 bp, Homo sapiens
tgcacacgcctctcctacaggcagcccagcaaatcatcga

SEQ ID NO: 774 - DNA, 40 bp, Homo sapiens
gagctggagaggaaggcgagaggcagctcgtcgggagcag

SEQ ID NO: 775 - DNA, 40 bp, Homo sapiens
gagctggagaggaaggcgaggcaggcactggtcgaccact

SEQ ID NO: 776 - DNA, 40 bp, Homo sapiens
ccgcctctgccttcggataggtctggccccaccctggagt

SEQ ID NO: 777 - DNA, 40 bp, Homo sapiens
ccgcctctgccttcggataggaaaggttgaaagagccaac

SEQ ID NO: 778 - DNA, 40 bp, Homo sapiens
tttctcatattgctcaacagttcttttttaggtatcatct

SEQ ID NO: 779 - DNA, 40 bp, Homo sapiens
tttctcatattgctcaacaggtatcatctttatcagaaag

SEQ ID NO: 780 - DNA, 40 bp, Homo sapiens
agtggctttggcgtcttatggaggcttgcttgcagagggg

SEQ ID NO: 781 - DNA, 40 bp, Homo sapiens
agtggctttggcgtcttatgggatggaggacgaaggttgg

SEQ ID NO: 782 - DNA, 40 bp, Homo sapiens
ggtgacactcaacttcacaggtctctccctctagtgccta

SEQ ID NO: 783 - DNA, 40 bp, Homo sapiens
ggtgacactcaacttcacagtgcctactggggccagaagc

SEQ ID NO: 784 - DNA, 40 bp, Homo sapiens
tttccattgggccaatcaagatgcctggaatgatgtcgtc

SEQ ID NO: 785 - DNA, 40 bp, Homo sapiens
gagggccaccaatgggacaaatgcctggaatgatgtcgtc

SEQ ID NO: 786 - DNA, 40 bp, Homo sapiens
agagacaaagagaagaaaaactcttactgttttacagtta

SEQ ID NO: 787 - DNA, 40 bp, Homo sapiens
agagacaaagagaagaaaaattaactctgctgtttgctgc

SEQ ID NO: 788 - DNA, 40 bp, Homo sapiens
ctcaccagcgccatcgtcagctctaggagttccagagcct

SEQ ID NO: 789 - DNA, 40 bp, Homo sapiens
ctcaccagcgccatcgtcagatggcaaggtcagccccggc

SEQ ID NO: 790 - DNA, 40 bp, Homo sapiens
atcaggtgctcatcctgaggtgtctgtctttaatacaggt

SEQ ID NO: 791 - DNA, 40 bp, Homo sapiens
atcaggtgctcatcctgagggtaatgcagagctctcagaa

SEQ ID NO: 792 - DNA, 40 bp, Homo sapiens
tctggcagcccacgatgctgcaagatggcatcgagcagca

SEQ ID NO: 793 - DNA, 40 bp, Homo sapiens
tctggcagcccacgatgctgggagtcgggctcacgtcctt

SEQ ID NO: 794 - DNA, 40 bp, Homo sapiens
agaattttaagatacttcagattttgtcttgtaggtttta

SEQ ID NO: 795 - DNA, 40 bp, Homo sapiens
agaattttaagatacttcaggttttatgggagaattgtag

SEQ ID NO: 796 - DNA, 40 bp, Homo sapiens
ccgcctctgccttcggataggctttatttaggtctggccc

SEQ ID NO: 797 - DNA, 40 bp, Homo sapiens
gagctagtcagactttagaggaaacagtactgctggagca

SEQ ID NO: 798 - DNA, 40 bp, Homo sapiens
aaattcttgaccaatctagggaaacagtactgctggagca

SEQ ID NO: 799 - DNA, 40 bp, Homo sapiens
cttcatctgtggataagcaggtcatgtcctccaggtttct

SEQ ID NO: 800 - DNA, 40 bp, Homo sapiens
cttcatctgtggataagcagtgcaggccaaggccccctgc

SEQ ID NO: 801 - DNA, 40 bp, Homo sapiens
agtatgggatattttaaaagattgttggaccttcagatgg

SEQ ID NO: 802 - DNA, 40 bp, Homo sapiens
tcattcttatttcaatgcagattgttggaccttcagatgg

SEQ ID NO: 803 - DNA, 40 bp, Homo sapiens
ctttatctgtgcatgaacagtgcaggccaaggccccctgc

SEQ ID NO: 804 - DNA, 40 bp, Homo sapiens
aagtcgtcctcttcagaaaggccggagcctcaacagaaag

SEQ ID NO: 805 - DNA, 40 bp, Homo sapiens
agagagaaacatccgaaaaagccggagcctcaacagaaag

SEQ ID NO: 806 - DNA, 40 bp, Homo sapiens
tgggctaccttaaccctggggtatttacacagagtcggcg

SEQ ID NO: 807 - DNA, 40 bp, Homo sapiens
tgggctaccttaaccctggggatttttgaccctcgtgtgg

SEQ ID NO: 808 - DNA, 40 bp, Homo sapiens
gactgccctaaaaggaaaagtttactgtttagactaaaga

SEQ ID NO: 809 - DNA, 40 bp, Homo sapiens
gactgccctaaaaggaaaagactaaagaagaaagacagtg

SEQ ID NO: 810 - DNA, 40 bp, Homo sapiens
tgatagttggagcggagactcataatggcagaacctgttt

SEQ ID NO: 811 - DNA, 40 bp, Homo sapiens
tgatagttggagcggagacttagcataatggcagaacctg

SEQ ID NO: 812 - DNA, 40 bp, Homo sapiens
tcattcttatttcaatgcagagacagggtcttgctctgtt

SEQ ID NO: 813 - DNA, 40 bp, Homo sapiens
tgacggtgccaccgcggcgcttttctcccttagatgcctt

SEQ ID NO: 814 - DNA, 40 bp, Homo sapiens
tgacggtgccaccgcggcgcagaggagtctgcaatgccga

SEQ ID NO: 815 - DNA, 40 bp, Homo sapiens
gcagtggctggagatcaaagtttcacccccagagggagcc

SEQ ID NO: 816 - DNA, 40 bp, Homo sapiens
gcagtggctggagatcaaagagagagtgtgcctattgact

SEQ ID NO: 817 - DNA, 40 bp, Homo sapiens
ggacgatggggatgagaaagatgacgaggaggataaagat

SEQ ID NO: 818 - DNA, 40 bp, Homo sapiens
ggacgatggggatgagaaagaagatgacgaggaggataaa

SEQ ID NO: 819 - DNA, 40 bp, Homo sapiens
actcttatgcagtccccatggactgaaccatcaagacacc

SEQ ID NO: 820 - DNA, 40 bp, Homo sapiens
gacccatgcatcctcctgtgctcctcccactgcagtgggc

SEQ ID NO: 821 - DNA, 40 bp, Homo sapiens
gacccatgcatcctcctgtgtgggcacagtggctcaggga

SEQ ID NO: 822 - DNA, 40 bp, Homo sapiens
catcaagcagctgttgcaatgtttagtcccaggaagcacc

SEQ ID NO: 823 - DNA, 40 bp, Homo sapiens
catcaagcagctgttgcaatctgcccacaaagaatccagc

SEQ ID NO: 824 - DNA, 40 bp, Homo sapiens
caatcattgacaatattatgaccctgcatgtgatggatca

SEQ ID NO: 825 - DNA, 40 bp, Homo sapiens
caatcattgacaatattatggaactgactcagcgcaagaa

SEQ ID NO: 826 - DNA, 40 bp, Homo sapiens
gggacactgtgccgaatgaacttgcttgccttttgtttta

SEQ ID NO: 827 - DNA, 40 bp, Homo sapiens
gggacactgtgccgaatgaacagctgcagtatctcggaag

SEQ ID NO: 828 - DNA, 40 bp, Homo sapiens
tcagggggcgcgtgctgaaggagctgcctgagttcgaggg

SEQ ID NO: 829 - DNA, 40 bp, Homo sapiens
tcgagccaggctgcaaaaaggagctgcctgagttcgaggg

SEQ ID NO: 830 - DNA, 40 bp, Homo sapiens
ctacaaccagagcgaggctgggtctcacaccctccaggga

SEQ ID NO: 831 - DNA, 40 bp, Homo sapiens
ctacaaccagagcgaggctgggaatgaatggctgcgacat

SEQ ID NO: 832 - DNA, 40 bp, Homo sapiens
tccaacaagcacctctgaagtcttctcattcacaggttaa

SEQ ID NO: 833 - DNA, 40 bp, Homo sapiens
tccaacaagcacctctgaaggttaaggctacctttccaga

SEQ ID NO: 834 - DNA, 40 bp, Homo sapiens
gttcccgaggctgtcaccagggtgttccctcaggtcaatg

SEQ ID NO: 835 - DNA, 40 bp, Homo sapiens
gttcccgaggctgtcaccagtggatactgaggctgtgtgg

SEQ ID NO: 836 - DNA, 40 bp, Homo sapiens
ccagatcaacacaattgatagtcgtactctttcagatgtc

SEQ ID NO: 837 - DNA, 40 bp, Homo sapiens
ccagatcaacacaattgataatgtcagcaatatttccaac

SEQ ID NO: 838 - DNA, 40 bp, Homo sapiens
cgtcctgcccccaactgccgctctgtcttccctgttccca

SEQ ID NO: 839 - DNA, 40 bp, Homo sapiens
cgtcctgcccccaactgccgcctctcagcgagaaggacac

SEQ ID NO: 840 - DNA, 40 bp, Homo sapiens
tgcagggggagcagcccaaggaggccccaccgccactgtc

SEQ ID NO: 841 - DNA, 40 bp, Homo sapiens
tgcagggggagcagcccaagccggccagccctgctgagga

SEQ ID NO: 842 - DNA, 40 bp, Homo sapiens
gactgccctaaaaggaaaagcagtttactgtttagactaa

SEQ ID NO: 843 - DNA, 40 bp, Homo sapiens
ctatgaggccatgactgcagtggatactgaggctgtgtgg

SEQ ID NO: 844 - DNA, 40 bp, Homo sapiens
cttctcaagatcagtctcaggtgccacgtgtgccaacgca

SEQ ID NO: 845 - DNA, 40 bp, Homo sapiens
cttctcaagatcagtctcaggaacctgacagaacttcaca

SEQ ID NO: 846 - DNA, 40 bp, Homo sapiens
accttaacaagatttatgagacttcctttaataagtgttg

SEQ ID NO: 847 - DNA, 40 bp, Homo sapiens
aatcactaggaactccagagacttcctttaataagtgttg

SEQ ID NO: 848 - DNA, 40 bp, Homo sapiens
actgggcttccaccgagcagaaacagcacttcttctcagt

SEQ ID NO: 849 - DNA, 40 bp, Homo sapiens
actgggcttccaccgagcaggagattacctggggcaattg

SEQ ID NO: 850 - DNA, 40 bp, Homo sapiens
ctgaagacgggattctttagctctccccacctggtgcagg

SEQ ID NO: 851 - DNA, 40 bp, Homo sapiens
ctgaagacgggattctttaggttcgggagcggatccgcat

SEQ ID NO: 852 - DNA, 40 bp, Homo sapiens
atctcaggagcacctgaatggtcccctgcctgtgcccttc

SEQ ID NO: 853 - DNA, 40 bp, Homo sapiens
cccaccccttcaccctgcaggtcccctgcctgtgcccttc

SEQ ID NO: 854 - DNA, 40 bp, Homo sapiens
ggccacacgcctctgccaagcccctctcccctggcacaga

SEQ ID NO: 855 - DNA, 40 bp, Homo sapiens
ggccacacgcctctgccaagacattgatgagtgtgagtct

SEQ ID NO: 856 - DNA, 40 bp, Homo sapiens
gagtacgaggtctccagcagcctgccctgtgcctacagcc

SEQ ID NO: 857 - DNA, 40 bp, Homo sapiens
gagtacgaggtctccagcagcctcgtgtgcatcaccgggg

SEQ ID NO: 858 - DNA, 40 bp, Homo sapiens
agcgcatcgcagcttccaagtacttcttcacagctcccct

SEQ ID NO: 859 - DNA, 40 bp, Homo sapiens
agcgcatcgcagcttccaaggctctcctccatcagtactt

SEQ ID NO: 860 - DNA, 40 bp, Homo sapiens
tgggcagccccccgcagacgttggtttttcagcagacctg

SEQ ID NO: 861 - DNA, 40 bp, Homo sapiens
tgggcagccccccgcagacgctcaacatcctggtggatac

SEQ ID NO: 862 - DNA, 40 bp, Homo sapiens
aaccaagaggacccacacaggatggtcttcacaggttctc

SEQ ID NO: 863 - DNA, 40 bp, Homo sapiens
aaccaagaggacccacacaggttctcaaagctggcccaga

SEQ ID NO: 864 - DNA, 40 bp, Homo sapiens
atattccttttatttctaagtcttttgtcttaggagttaa

SEQ ID NO: 865 - DNA, 40 bp, Homo sapiens
atattccttttatttctaaggagttaaacatagatgtagc

SEQ ID NO: 866 - DNA, 40 bp, Homo sapiens
ggtcctgaacgctgtgaaataacttcgcccccagcttcaa

SEQ ID NO: 867 - DNA, 40 bp, Homo sapiens
ggtcctgaacgctgtgaaattgtactgtcagaacttcgcc

SEQ ID NO: 868 - DNA, 40 bp, Homo sapiens
tggagcagtatgccagcaagacttttcccccaggttcttc

SEQ ID NO: 869 - DNA, 40 bp, Homo sapiens
tggagcagtatgccagcaaggttcttcatgacagccagat

SEQ ID NO: 870 - DNA, 40 bp, Homo sapiens
tcgtgcagaccctggagaagatctcacagatgtgcagtct

SEQ ID NO: 871 - DNA, 40 bp, Homo sapiens
tcgtgcagaccctggagaagcatggcttcagtgatattaa

SEQ ID NO: 872 - DNA, 40 bp, Homo sapiens
ttgaagctcagtgagaaaagttcttctgtttatgtcttcc

SEQ ID NO: 873 - DNA, 40 bp, Homo sapiens
ttgaagctcagtgagaaaaggatgatggagatagccaaag

SEQ ID NO: 874 - DNA, 40 bp, Homo sapiens
cgccctgacacacaatcaggacttctctatctacaggctc

SEQ ID NO: 875 - DNA, 40 bp, Homo sapiens
cgccctgacacacaatcagggctctgttgcaagagggggt

SEQ ID NO: 876 - DNA, 40 bp, Homo sapiens
ttgctggccatcggattgggcccttcgtttcaggatggat

SEQ ID NO: 877 - DNA, 40 bp, Homo sapiens
ttgctggccatcggattggggatctatattggaaggcgtc

SEQ ID NO: 878 - DNA, 40 bp, Homo sapiens
ccattcgagagcatcagaagattgggaggaaggaccggct

SEQ ID NO: 879 - DNA, 40 bp, Homo sapiens
ccattcgagagcatcagaagctaaaccatttcccaggctc

SEQ ID NO: 880 - DNA, 40 bp, Homo sapiens
tcaggagcagagaggaaaagtgcatttgcccagtataaca

SEQ ID NO: 881 - DNA, 40 bp, Homo sapiens
ctcagggaaggggcagcacatgcatttgcccagtataaca

SEQ ID NO: 882 - DNA, 40 bp, Homo sapiens
gtgtggcaagtactttcaagtatctgcccttctattacag

SEQ ID NO: 883 - DNA, 40 bp, Homo sapiens
gtgtggcaagtactttcaaggccggggtttgaagtctcac

SEQ ID NO: 884 - DNA, 40 bp, Homo sapiens
aaaatcattgattcccttgaaattctctttactctacctt

SEQ ID NO: 885 - DNA, 40 bp, Homo sapiens
aaaatcattgattcccttgagtggttagacgatgctatta

SEQ ID NO: 886 - DNA, 40 bp, Homo sapiens
tgctcagaggtgctttgaagcccatccacaacctgctcat

SEQ ID NO: 887 - DNA, 40 bp, Homo sapiens
tgctcagaggtgctttgaagatgccggaggccccgcctct

SEQ ID NO: 888 - DNA, 40 bp, Homo sapiens
ccacggccacggccgcatagctttgtattcctgcaggcaa

SEQ ID NO: 889 - DNA, 40 bp, Homo sapiens
ccacggccacggccgcataggcaagcaccggaagcacccc

SEQ ID NO: 890 - DNA, 40 bp, Homo sapiens
catgccggggccagaggatggctctttccacctgtctgca

SEQ ID NO: 891 - DNA, 40 bp, Homo sapiens
catgccggggccagaggatgctctgcacccgggacagtga

SEQ ID NO: 892 - DNA, 40 bp, Homo sapiens
ggccaagcaagaacaaaaagtattttcttctaggatggaa

SEQ ID NO: 893 - DNA, 40 bp, Homo sapiens
ggccaagcaagaacaaaaagtgaaatgcaaaatggaggac

SEQ ID NO: 894 - DNA, 40 bp, Homo sapiens
gaagaacaggatattaatagtatgtttttgtttttaggag

SEQ ID NO: 895 - DNA, 40 bp, Homo sapiens
gaagaacaggatattaataggaggattctctatgggagga

SEQ ID NO: 896 - DNA, 40 bp, Homo sapiens
caattcagtagattcaccctcaacatctgaatgaattgat

SEQ ID NO: 897 - DNA, 40 bp, Homo sapiens
aggtcttcctggacctggagcaacatctgaatgaattgat

SEQ ID NO: 898 - DNA, 40 bp, Homo sapiens
agagggcacgggacatccagcccctctgcccctgcaggag

SEQ ID NO: 899 - DNA, 40 bp, Homo sapiens
agagggcacgggacatccaggaggccgtggagtcctgcct

SEQ ID NO: 900 - DNA, 40 bp, Homo sapiens
agatgattgaggcagccaagctcttttctgtcttcttggt

SEQ ID NO: 901 - DNA, 40 bp, Homo sapiens
agatgattgaggcagccaaggccgtctatacccaggattg

SEQ ID NO: 902 - DNA, 40 bp, Homo sapiens
gctgctctcttcaatacaagtgcttctgcttccaggatac

SEQ ID NO: 903 - DNA, 40 bp, Homo sapiens
gctgctctcttcaatacaaggataccaagggttcgagttt

SEQ ID NO: 904 - DNA, 40 bp, Homo sapiens
aatagaacttccaactactggccctttttcagtaaagtca

SEQ ID NO: 905 - DNA, 40 bp, Homo sapiens
aatagaacttccaactactgtaaagtcatcacctggcctt

SEQ ID NO: 906 - DNA, 40 bp, Homo sapiens
tgttactgcagtggctacaggtctctctcttgcaggtggt

SEQ ID NO: 907 - DNA, 40 bp, Homo sapiens
tgttactgcagtggctacaggtggtcctgacaaccaagtc

SEQ ID NO: 908 - DNA, 40 bp, Homo sapiens
acatcacaaagcaacctgtggggttttgtttttgttttag

SEQ ID NO: 909 - DNA, 40 bp, Homo sapiens
acatcacaaagcaacctgtggtgtacctgaaggaaatctt

SEQ ID NO: 910 - DNA, 40 bp, Homo sapiens
ggtgctggctgcctgcgaaaccctggctgcccctgcaggc

SEQ ID NO: 911 - DNA, 40 bp, Homo sapiens
ggtgctggctgcctgcgaaagcctgctcaccagccgccag

SEQ ID NO: 912 - DNA, 40 bp, Homo sapiens
cctctctgctcgagaaggagtgtgtgtctttttgccaaca

SEQ ID NO: 913 - DNA, 40 bp, Homo sapiens
cctctctgctcgagaaggagctggagcagagccagaagga

SEQ ID NO: 914 - DNA, 40 bp, Homo sapiens
ctggaagctcaaggtactagatttttcctctctctgtctt

SEQ ID NO: 915 - DNA, 40 bp, Homo sapiens
ctggaagctcaaggtactagtttgccaaagaaactagagt

SEQ ID NO: 916 - DNA, 40 bp, Homo sapiens
cggcgatgactcggacccagcttctctccacagggctcct

SEQ ID NO: 917 - DNA, 40 bp, Homo sapiens
cggcgatgactcggacccagggctccttcagtggtagatg

SEQ ID NO: 918 - DNA, 40 bp, Homo sapiens
ccgccaggagaacaagcccatcccctcacaggcagagata

SEQ ID NO: 919 - DNA, 40 bp, Homo sapiens
ccgccaggagaacaagcccaagttagtcccctcacaggca

SEQ ID NO: 920 - DNA, 40 bp, Homo sapiens
cagcagcagctctgcttgagctactgccaacaccactgct

SEQ ID NO: 921 - DNA, 40 bp, Homo sapiens
cagcagcagctctgcttgaggtgttggatcctgaacaaaa

SEQ ID NO: 922 - DNA, 40 bp, Homo sapiens
gcacttatggtggtggcgtgagtttccagaccttcagcat

SEQ ID NO: 923 - DNA, 40 bp, Homo sapiens
gcacttatggtggtggcgtgcacctgtccagcccactggc

SEQ ID NO: 924 - DNA, 40 bp, Homo sapiens
gtggctccagtatcagaaagagaccacagagctgggcagc

SEQ ID NO: 925 - DNA, 40 bp, Homo sapiens
gacctgctcaagttcactcaagaccacagagctgggcagc

SEQ ID NO: 926 - DNA, 40 bp, Homo sapiens
tgtgggcatggagcgaaaagtgctgccctgctttctctgt

SEQ ID NO: 927 - DNA, 40 bp, Homo sapiens
tgtgggcatggagcgaaaagggtgtgctgtccgacctcac

SEQ ID NO: 928 - DNA, 40 bp, Homo sapiens
ttcctcttcccctcatcaagtcctctctttctcctttgtc

SEQ ID NO: 929 - DNA, 40 bp, Homo sapiens
ttcctcttcccctcatcaagagctatctgttccagctgct

SEQ ID NO: 930 - DNA, 40 bp, Homo sapiens
ggggcactgacacggctactagcctctctggcctcttcca

SEQ ID NO: 931 - DNA, 40 bp, Homo sapiens
ggggcactgacacggctactgtgttggacatggccacgga

SEQ ID NO: 932 - DNA, 40 bp, Homo sapiens
aggctgtagcaggactccagggttgggaagaacatggaaa

SEQ ID NO: 933 - DNA, 40 bp, Homo sapiens
aggctgtagcaggactccaggaagatgttaccgagtactt

SEQ ID NO: 934 - DNA, 40 bp, Homo sapiens
ccgaggatgctaaggggcagtttctgttccaggtgaaatc

SEQ ID NO: 935 - DNA, 40 bp, Homo sapiens
ccgaggatgctaaggggcaggattggatagctttagtcaa

SEQ ID NO: 936 - DNA, 40 bp, Homo sapiens
gcctcccggtccgcaagcagaatgaagaactgcatgtggc

SEQ ID NO: 937 - DNA, 40 bp, Homo sapiens
gcctcccggtccgcaagcagttccagttatactccgtgta

SEQ ID NO: 938 - DNA, 40 bp, Homo sapiens
tcgtaacaggggttgcacaggtgaagatcatgacggagaa

SEQ ID NO: 939 - DNA, 40 bp, Homo sapiens
ctgtgacgggtgtcgcccaggtgaagatcatgacggagaa

SEQ ID NO: 940 - DNA, 40 bp, Homo sapiens
gtttggggaagtatggatggagaaagctgatggtttgtgt

SEQ ID NO: 941 - DNA, 40 bp, Homo sapiens
gtttggggaagtatggatgggtacctggaatggaaacaca

SEQ ID NO: 942 - DNA, 40 bp, Homo sapiens
taactaatccttctcagcagaaagagctgggctccactga

SEQ ID NO: 943 - DNA, 40 bp, Homo sapiens
cagcctaccagaggcaccagaaagagctgggctccactga

SEQ ID NO: 944 - DNA, 40 bp, Homo sapiens
cctgcgcaactggtaccgaggcgcagccagtgtctttgga

SEQ ID NO: 945 - DNA, 40 bp, Homo sapiens
cctgcgcaactggtaccgaggggacaaccccaacaagccc

SEQ ID NO: 946 - DNA, 40 bp, Homo sapiens
ataaaaattgcttagtaaagatttttgccttctctcaggt

SEQ ID NO: 947 - DNA, 40 bp, Homo sapiens
ataaaaattgcttagtaaaggtcaaagattctaaactgcc

SEQ ID NO: 948 - DNA, 40 bp, Homo sapiens
tgagttcatggatgatgccaaaattctttttaatctttcg

SEQ ID NO: 949 - DNA, 40 bp, Homo sapiens
tgagttcatggatgatgccaacatgtgcattgccattgcg

SEQ ID NO: 950 - DNA, 40 bp, Homo sapiens
agagttgaaaaacactggcgtctccttttcaggaatcaca

SEQ ID NO: 951 - DNA, 40 bp, Homo sapiens
agagttgaaaaacactggcgtttaattggttggggtcaga

SEQ ID NO: 952 - DNA, 40 bp, Homo sapiens
tggggccacaaagacagatgctggatacacagtatcgtcg

SEQ ID NO: 953 - DNA, 40 bp, Homo sapiens
tggggccacaaagacagatgaaaccccatggcgactctag

SEQ ID NO: 954 - DNA, 40 bp, Homo sapiens
aacatggaatcatcaggaagttctccatttctatttagcc

SEQ ID NO: 955 - DNA, 40 bp, Homo sapiens
aacatggaatcatcaggaagccaaggtggaagagcacctt

SEQ ID NO: 956 - DNA, 40 bp, Homo sapiens
cgtgcgtgtgtgtgctcttgctatacacagaatgggattt

SEQ ID NO: 957 - DNA, 40 bp, Homo sapiens
cttaggaaagacaaagaactctatacacagaatgggattt

SEQ ID NO: 958 - DNA, 40 bp, Homo sapiens
cccagcctgctgtccagcagcctcttgcactgtaccccca

SEQ ID NO: 959 - DNA, 40 bp, Homo sapiens
cccagcctgctgtccagcaggcccccacccccgctgcccc

SEQ ID NO: 960 - DNA, 40 bp, Homo sapiens
acccaaggctcgtcctgaagtttctctgtttccttctgca

SEQ ID NO: 961 - DNA, 40 bp, Homo sapiens
acccaaggctcgtcctgaagacgtggttaacttggacctc

SEQ ID NO: 962 - DNA, 40 bp, Homo sapiens
gaacccggtggtacccatagttgctttgtcccctcctcag

SEQ ID NO: 963 - DNA, 40 bp, Homo sapiens
gaacccggtggtacccataggttgcctggccacggcggcc

SEQ ID NO: 964 - DNA, 40 bp, Homo sapiens
aatggaagtaccagcagaagaattttatttttttcaagat

SEQ ID NO: 965 - DNA, 40 bp, Homo sapiens
aatggaagtaccagcagaagattctactcaacatgtccct

SEQ ID NO: 966 - DNA, 40 bp, Homo sapiens
ggcagctgttagccgagcaagagctggacgaggtattgtg

SEQ ID NO: 967 - DNA, 40 bp, Homo sapiens
ggcagctgttagccgagcaacttgctgatgaccgtatggc

SEQ ID NO: 968 - DNA, 40 bp, Homo sapiens
gtttagaaatggaaaaatgttttttgcttttacagtaaca

SEQ ID NO: 969 - DNA, 40 bp, Homo sapiens
gtttagaaatggaaaaatgttaacaaatgtggcaattatt

SEQ ID NO: 970 - DNA, 40 bp, Homo sapiens
aaatctcgtggacttctaagttttctgtttgcccagaaag

SEQ ID NO: 971 - DNA, 40 bp, Homo sapiens
aaatctcgtggacttctaagaaagcgccatggcctgtgct

SEQ ID NO: 972 - DNA, 40 bp, Homo sapiens
agttccggggctacctgatgccttcctctttgcagaaatc

SEQ ID NO: 973 - DNA, 40 bp, Homo sapiens
agttccggggctacctgatgaaatctctccagacctcgct

SEQ ID NO: 974 - DNA, 40 bp, Homo sapiens
aagaaggaatccacgttctagtcatttcttttcaggattg

SEQ ID NO: 975 - DNA, 40 bp, Homo sapiens
aagaaggaatccacgttctagattggccatttgatgatgg

SEQ ID NO: 976 - DNA, 40 bp, Homo sapiens
cgctggcaccatgaacccaggaccaagtgagcagagagaa

SEQ ID NO: 977 - DNA, 40 bp, Homo sapiens
agcccctgcttgacaaccagtttcatgtcccaccaggttg

SEQ ID NO: 978 - DNA, 40 bp, Homo sapiens
agcccctgcttgacaaccaggttggttttaagaacatgca

SEQ ID NO: 979 - DNA, 40 bp, Homo sapiens
ttggctgtaggaaactcagggtccagctgtagttcctctg

SEQ ID NO: 980 - DNA, 40 bp, Homo sapiens
ttggctgtaggaaactcaggcggcgttgacattccccagg

SEQ ID NO: 981 - DNA, 40 bp, Homo sapiens
tgtatctccgacactcagagactgtctctggaggttatga

SEQ ID NO: 982 - DNA, 40 bp, Homo sapiens
tgtatctccgacactcagaggatttccctagagattatga

SEQ ID NO: 983 - DNA, 40 bp, Homo sapiens
aggctgatctactgcaggagccacgtcatgaatattttaa

SEQ ID NO: 984 - DNA, 40 bp, Homo sapiens
aggctgatctactgcaggaggaagctgaaaccccacgtag

SEQ ID NO: 985 - DNA, 40 bp, Homo sapiens
gctcagccccctccccacagggcccctagaagcctgtttc

SEQ ID NO: 986 - DNA, 40 bp, Homo sapiens
tgaccctgcagctcctcaaaggcccctagaagcctgtttc

SEQ ID NO: 987 - DNA, 40 bp, Homo sapiens
gccgacccgcctgcgacgctcttttcttgcctggagaaga

SEQ ID NO: 988 - DNA, 40 bp, Homo sapiens
gccgacccgcctgcgacgctgggaccgtgatgcccggccc

SEQ ID NO: 989 - DNA, 40 bp, Homo sapiens
tgcggagaccccttcgggaggtgacagttcgtgatgctat

SEQ ID NO: 990 - DNA, 40 bp, Homo sapiens
tgcggagaccccttcgggaggtctccgggctgctgaagag

SEQ ID NO: 991 - DNA, 40 bp, Homo sapiens
ctatcagtaggtttttagagatgaacatcactcgaaaact

SEQ ID NO: 992 - DNA, 40 bp, Homo sapiens
gcattgatgtggaagatgcaatgaacatcactcgaaaact

SEQ ID NO: 993 - DNA, 40 bp, Homo sapiens
gcattgatgtggaagatgcagtttttttcctggcagaaga

SEQ ID NO: 994 - DNA, 40 bp, Homo sapiens
cagtgggcggatgacatttggtacagcctcggaactggct

SEQ ID NO: 995 - DNA, 40 bp, Homo sapiens
cagtgggcggatgacatttgccctctgttgctattctttg

SEQ ID NO: 996 - DNA, 40 bp, Homo sapiens
ggtgtccatggcctgcactcctatacctttctgccgtgta

SEQ ID NO: 997 - DNA, 40 bp, Homo sapiens
ggtgtccatggcctgcactcttacgaaaagcggctgtact

SEQ ID NO: 998 - DNA, 40 bp, Homo sapiens
actgggaagttcttaaaaagtccccctctacacaagaatc

SEQ ID NO: 999 - DNA, 40 bp, Homo sapiens
actgggaagttcttaaaaaggttcacagatgaagagtcta

SEQ ID NO: 1000 - DNA, 40 bp, Homo sapiens
gctgagcggggcgacccgagtcttctcattcacaggttaa

SEQ ID NO: 1001 - DNA, 40 bp, Homo sapiens
tgttccacctcctcctgcagctcccccttttcttccagtg

SEQ ID NO: 1002 - DNA, 40 bp, Homo sapiens
tgttccacctcctcctgcagtgggccggatgtatcccccg

SEQ ID NO: 1003 - DNA, 40 bp, Homo sapiens
acccatgagaatgctcagagctatgaagaccccgcggccc

SEQ ID NO: 1004 - DNA, 40 bp, Homo sapiens
ctggcccctgagatccgcagctatgaagaccccgcggccc

SEQ ID NO: 1005 - DNA, 40 bp, Homo sapiens
caagctcgagtccatcgatgaacccatctgcgccgtcggc

SEQ ID NO: 1006 - DNA, 40 bp, Homo sapiens
caagctcgagtccatcgatggtgcccggtaccatgccctc

SEQ ID NO: 1007 - DNA, 40 bp, Homo sapiens
cttcactgtcaccgtcacagaacccccagtgcggatcata

SEQ ID NO: 1008 - DNA, 40 bp, Homo sapiens
cttcactgtcaccgtcacagagtcttaccaaagtcaggac

SEQ ID NO: 1009 - DNA, 40 bp, Homo sapiens
agaaacagaaaccagcacaggatgtacctggcaaagattc

SEQ ID NO: 1010 - DNA, 40 bp, Homo sapiens
agaaacagaaaccagcacagaattatgatgacaatttcaa

SEQ ID NO: 1011 - DNA, 40 bp, Homo sapiens
ttctgcatctgtgggccgagtgatcctgccatgaagcagt

SEQ ID NO: 1012 - DNA, 40 bp, Homo sapiens
aaaggagtgcttatagaatgtgatcctgccatgaagcagt

SEQ ID NO: 1013 - DNA, 40 bp, Homo sapiens
aggatcggcaacatggcaaggcctctactacgtggacagt

SEQ ID NO: 1014 - DNA, 40 bp, Homo sapiens
ctgggataagagaggccctggcctctactacgtggacagt

SEQ ID NO: 1015 - DNA, 40 bp, Homo sapiens
gttcaggacacaataagcaggttgcagagcctgaggcctg

SEQ ID NO: 1016 - DNA, 40 bp, Homo sapiens
gggagggagagaatacccaggttgcagagcctgaggcctg

SEQ ID NO: 1017 - DNA, 40 bp, Homo sapiens
tacccggatgatggcatgggaagttcttgctgtctttcag

SEQ ID NO: 1018 - DNA, 40 bp, Homo sapiens
tacccggatgatggcatggggtatggcgactacccgaagc

SEQ ID NO: 1019 - DNA, 40 bp, Homo sapiens
gacatatgagtcaaaggaagcccggtggcgcctgtccgtc

SEQ ID NO: 1020 - DNA, 40 bp, Homo sapiens
gacatatgagtcaaaggaagaagcccggtggcgcctgtcc

SEQ ID NO: 1021 - DNA, 40 bp, Homo sapiens
cggatcaacttcgacaaatagtggttgttacctcttccta

SEQ ID NO: 1022 - DNA, 40 bp, Homo sapiens
cggatcaacttcgacaaataccacccaggctactttggga

SEQ ID NO: 1023 - DNA, 40 bp, Homo sapiens
ttataggcgtgatgatagagtttcatttaacttaggtccc

SEQ ID NO: 1024 - DNA, 40 bp, Homo sapiens
ttataggcgtgatgatagaggtcccccccaaagacccaaa

SEQ ID NO: 1025 - DNA, 40 bp, Homo sapiens
tggaaatatttctagacttggtgtcagttgtacccgaggc

SEQ ID NO: 1026 - DNA, 40 bp, Homo sapiens
tcggcccagaagaaccccgcctatacacagaatgggattt

SEQ ID NO: 1027 - DNA, 40 bp, Homo sapiens
gctgaagggaaaagacaccaaaacacaaacagcagaatgg

SEQ ID NO: 1028 - DNA, 40 bp, Homo sapiens
gctgaagggaaaagacaccagttgcctggcagagcagtgg

SEQ ID NO: 1029 - DNA, 40 bp, Homo sapiens
catcatcaagtttttcaatgacgagctggtccagccatcc

SEQ ID NO: 1030 - DNA, 40 bp, Homo sapiens
catcatcaagtttttcaatgaacgtgctgagcatcacgat

SEQ ID NO: 1031 - DNA, 40 bp, Homo sapiens
gagggcctgctcattcaaagatgttctcagtgcagctgag

SEQ ID NO: 1032 - DNA, 40 bp, Homo sapiens
acatgcttcaaataaatcagatgttctcagtgcagctgag

SEQ ID NO: 1033 - DNA, 40 bp, Homo sapiens
ctgaggctaatgaaaaacagggaagctgccaaagaatgtc

SEQ ID NO: 1034 - DNA, 40 bp, Homo sapiens
ctgaggctaatgaaaaacagggaagctgcccgggagtgtc

SEQ ID NO: 1035 - DNA, 40 bp, Homo sapiens
cggctgggactcttccatgcgtggcactggaagcagactg

SEQ ID NO: 1036 - DNA, 40 bp, Homo sapiens
cggctgggactcttccatgcagttgaaactggttgacaac

SEQ ID NO: 1037 - DNA, 40 bp, Homo sapiens
agtgaatgtagttgcaccagtgacaatacttgtatggagt

SEQ ID NO: 1038 - DNA, 40 bp, Homo sapiens
agtgaatgtagttgcaccaggatttgtacacacagatatg

SEQ ID NO: 1039 - DNA, 40 bp, Homo sapiens
attcacacagagccacctaggccaggctaccaacgtcttt

SEQ ID NO: 1040 - DNA, 40 bp, Homo sapiens
tgaggatcaatcctggggaggccaggctaccaacgtcttt

SEQ ID NO: 1041 - DNA, 40 bp, Homo sapiens
tggaaaagtataaaggcaaaattcttcaaagaaggaacca

SEQ ID NO: 1042 - DNA, 40 bp, Homo sapiens
tggaaaagtataaaggcaaagtttcactagttgtaaacgt

SEQ ID NO: 1043 - DNA, 40 bp, Homo sapiens
atactaagaacaacaatttgaatgggacaacagaagaagt

SEQ ID NO: 1044 - DNA, 40 bp, Homo sapiens
atactaagaacaacaatttgcttcgtcagcaattgaagtg

SEQ ID NO: 1045 - DNA, 40 bp, Homo sapiens
tggccttgacctccaaccaggtcctgcacccagacctcac

SEQ ID NO: 1046 - DNA, 40 bp, Homo sapiens
tggccttgacctccaaccaggagtacctggacctgtccat

SEQ ID NO: 1047 - DNA, 40 bp, Homo sapiens
tccttgaacactacaattagacctcttcttgggtgaattt

SEQ ID NO: 1048 - DNA, 40 bp, Homo sapiens
tccttgaacactacaattagctgttctgaagcccagaaaa

SEQ ID NO: 1049 - DNA, 40 bp, Homo sapiens
acaccattgaggagatccaggtgcggcagctggtgcctcg

SEQ ID NO: 1050 - DNA, 40 bp, Homo sapiens
acaccattgaggagatccagggactgaccacagcccatga

SEQ ID NO: 1051 - DNA, 40 bp, Homo sapiens
cccatgtataaggctttccggatgtgctctttgtcctcca

SEQ ID NO: 1052 - DNA, 40 bp, Homo sapiens
cccatgtataaggctttccggagtgacagttcattcaatt

SEQ ID NO: 1053 - DNA, 40 bp, Homo sapiens
ctcccagtgctgtatatcccggaattcctggggaagtcgg

SEQ ID NO: 1054 - DNA, 40 bp, Homo sapiens
gagctgccacggatactgagggaattcctggggaagtcgg

SEQ ID NO: 1055 - DNA, 40 bp, Homo sapiens
ggatgcgcgtctggtcaagggctgcagagaaggctggtat

SEQ ID NO: 1056 - DNA, 40 bp, Homo sapiens
agccgcagagcatcctggcggctgcagagaaggctggtat

SEQ ID NO: 1057 - DNA, 40 bp, Homo sapiens
acatgcttcaaataaatcagcttctctccaagataaaatg

SEQ ID NO: 1058 - DNA, 40 bp, Homo sapiens
aacaaagaaataattcacaggatgaagatgggtttcaaga

SEQ ID NO: 1059 - DNA, 40 bp, Homo sapiens
ctgagtctttatattttgaggatgaagatgggtttcaaga

SEQ ID NO: 1060 - DNA, 40 bp, Homo sapiens
tagccaccactgtgtgccagggatatcttctaaccatacc

SEQ ID NO: 1061 - DNA, 40 bp, Homo sapiens
gggaaaagtctttcaccctgggatatcttctaaccatacc

SEQ ID NO: 1062 - DNA, 40 bp, Homo sapiens
cctaccagccacttcgggaggtatcagagtgctccatctc

SEQ ID NO: 1063 - DNA, 40 bp, Homo sapiens
cctaccagccacttcgggaggtattgccagggaacagacg

SEQ ID NO: 1064 - DNA, 40 bp, Homo sapiens
gtcccggcttccccctactcgcctggctcagaatctaacc

SEQ ID NO: 1065 - DNA, 40 bp, Homo sapiens
gtcccggcttccccctactcagtgaagaagccaccctcag

SEQ ID NO: 1066 - DNA, 40 bp, Homo sapiens
cttaagcatatatttaaagggtgaagatgcttttgatgcc

SEQ ID NO: 1067 - DNA, 40 bp, Homo sapiens
cttaagcatatatttaaagggagatgtttttgattcagcc

SEQ ID NO: 1068 - DNA, 40 bp, Homo sapiens
caggaacaagtatctgacagaaaatatctttcaggcctgg

SEQ ID NO: 1069 - DNA, 40 bp, Homo sapiens
caggaacaagtatctgacagtcaagtcctaattcgaagca

SEQ ID NO: 1070 - DNA, 40 bp, Homo sapiens
gaagttctgaggaaaagcagaatgctgtgtcctctgaaga

SEQ ID NO: 1071 - DNA, 40 bp, Homo sapiens
gaagttctgaggaaaagcagctttacaacaaatacccaga

SEQ ID NO: 1072 - DNA, 40 bp, Homo sapiens
atctccctcttggtgtacaaattgttttcagaaaacacaa

SEQ ID NO: 1073 - DNA, 40 bp, Homo sapiens
atctccctcttggtgtacaaaaaacacaaggaatacaacc

SEQ ID NO: 1074 - DNA, 40 bp, Homo sapiens
tgcgagtactgcttcaccagaaagaagattggcccatgca

SEQ ID NO: 1075 - DNA, 40 bp, Homo sapiens
tgcgagtactgcttcaccaggaaagaaggattgtccaaat

SEQ ID NO: 1076 - DNA, 40 bp, Homo sapiens
tccagaaagtgaaactaaaattttaatccaggtgctggtt

SEQ ID NO: 1077 - DNA, 40 bp, Homo sapiens
tccagaaagtgaaactaaaagagcgtcaggaagcagagaa

SEQ ID NO: 1078 - DNA, 40 bp, Homo sapiens
agattctacagataaatcagatttcggaaacttctggcag

SEQ ID NO: 1079 - DNA, 40 bp, Homo sapiens
agattctacagataaatcagctgcacttagtgcattggaa

SEQ ID NO: 1080 - DNA, 40 bp, Homo sapiens
tggctggcttcagtggaccaaattttcaggatggctgtat

SEQ ID NO: 1081 - DNA, 40 bp, Homo sapiens
tggctggcttcagtggaccagccttcatggtgaaacacct

SEQ ID NO: 1082 - DNA, 40 bp, Homo sapiens
ccctgctcatcacctacggggaacccagaatgggggcttc

SEQ ID NO: 1083 - DNA, 40 bp, Homo sapiens
ggcagccaccacgggctcggacaatttatgaaaaccgaat

SEQ ID NO: 1084 - DNA, 40 bp, Homo sapiens
tgataattgggcctccaagaacaatttatgaaaaccgaat

SEQ ID NO: 1085 - DNA, 40 bp, Homo sapiens
accgccctgcactgctacaggagtcctccgctctgccaca

SEQ ID NO: 1086 - DNA, 40 bp, Homo sapiens
accgccctgcactgctacaggaagggcctgaccttcgtct

SEQ ID NO: 1087 - DNA, 40 bp, Homo sapiens
tcacaattataggggaagagctcgtggtctgggttgatcc

SEQ ID NO: 1088 - DNA, 40 bp, Homo sapiens
gtgctattaaagaagaagatctcgtggtctgggttgatcc

SEQ ID NO: 1089 - DNA, 40 bp, Homo sapiens
ctcgtctatgatatcaccagatgcccgaatgctagcgagc

SEQ ID NO: 1090 - DNA, 40 bp, Homo sapiens
ctcgtctatgatatcaccagccgagaaacctacaatgcgc

SEQ ID NO: 1091 - DNA, 40 bp, Homo sapiens
caatgccacagggcaggctggaaggctgggatgcatggga

SEQ ID NO: 1092 - DNA, 40 bp, Homo sapiens
caatgccacagggcaggctgactgcaaagcccaggatgag

SEQ ID NO: 1093 - DNA, 40 bp, Homo sapiens
tcagaagagaaaatcggatgacaggcggacccacaggccc

SEQ ID NO: 1094 - DNA, 40 bp, Homo sapiens
tcagaagagaaaatcggatggaccttgaccctgctgttca

SEQ ID NO: 1095 - DNA, 40 bp, Homo sapiens
tgactgccgctttctctcaggcccggaaacaaaactcatg

SEQ ID NO: 1096 - DNA, 40 bp, Homo sapiens
ctaaagccttctataaaactgcccggaaacaaaactcatg

SEQ ID NO: 1097 - DNA, 40 bp, Homo sapiens
atgcagatacacaaagcaagccatgcagtttggtcagctc

SEQ ID NO: 1098 - DNA, 40 bp, Homo sapiens
atgcagatacacaaagcaaggtgcaccagctatatgaaac

SEQ ID NO: 1099 - DNA, 40 bp, Homo sapiens
tactgatcatattgtccaagtcaaagtaaacaagtatgga

SEQ ID NO: 1100 - DNA, 40 bp, Homo sapiens
aagagtgccaaaaaaagaagtcaaagtaaacaagtatgga

SEQ ID NO: 1101 - DNA, 40 bp, Homo sapiens
tgtcatccattgtggaagagccccgaaacacagcagagct

SEQ ID NO: 1102 - DNA, 40 bp, Homo sapiens
tgtcatccattgtggaagagctgctggatcagtgcctggc

SEQ ID NO: 1103 - DNA, 40 bp, Homo sapiens
taccggaaacctaggaaaaggcgccaagcccatctttgtg

SEQ ID NO: 1104 - DNA, 40 bp, Homo sapiens
gctgccaaagccttagacaagcgccaagcccatctttgtg

SEQ ID NO: 1105 - DNA, 40 bp, Homo sapiens
aggatatcggtttcattaagaaagacctgagctgtcttcc

SEQ ID NO: 1106 - DNA, 40 bp, Homo sapiens
aggatatcggtttcattaagttggactaaatgctcttcct

SEQ ID NO: 1107 - DNA, 40 bp, Homo sapiens
gcggcgggcagtggcggcaggtgtacatttttatctttca

SEQ ID NO: 1108 - DNA, 40 bp, Homo sapiens
gcggcgggcagtggcggcagaatgttggctaccagggtat

SEQ ID NO: 1109 - DNA, 40 bp, Homo sapiens
tatccagcactgaccacatggacagacgttgaaagatacc

SEQ ID NO: 1110 - DNA, 40 bp, Homo sapiens
cctgattctccccaccagaggacagacgttgaaagatacc

SEQ ID NO: 1111 - DNA, 40 bp, Homo sapiens
ttcatcatggtgtggtggagctctcctcttgtttttcagg

SEQ ID NO: 1112 - DNA, 40 bp, Homo sapiens
ttcatcatggtgtggtggaggttgacgccgctgtcacccc

SEQ ID NO: 1113 - DNA, 40 bp, Homo sapiens
tgaaatcagaaaaaaatatgtttattttgtttcaggcctg

SEQ ID NO: 1114 - DNA, 40 bp, Homo sapiens
tgaaatcagaaaaaaatatggcctgtttaaagaagaaaac

SEQ ID NO: 1115 - DNA, 40 bp, Homo sapiens
gcaaggatatataataactgctgctttatttttccacaga

SEQ ID NO: 1116 - DNA, 40 bp, Homo sapiens
gcaaggatatataataactgattggtgtgcccgtttaata

SEQ ID NO: 1117 - DNA, 40 bp, Homo sapiens
gaactgcaaaggcttcagaggatttgtacacacagatatg

SEQ ID NO: 1118 - DNA, 40 bp, Homo sapiens
ttggagatcaggacgcaaaggtcaccatcagaaaagctaa

SEQ ID NO: 1119 - DNA, 40 bp, Homo sapiens
gatctggattctcgtttcaggtcaccatcagaaaagctaa

SEQ ID NO: 1120 - DNA, 40 bp, Homo sapiens
tggaagaggctacctctggggtcaatgagagtgaaatggc

SEQ ID NO: 1121 - DNA, 40 bp, Homo sapiens
tggaagaggctacctctggggtaacccccgggactttgcc

SEQ ID NO: 1122 - DNA, 40 bp, Homo sapiens
tctggagccatacgtgacagtgacctgaccaacggtgcag

SEQ ID NO: 1123 - DNA, 40 bp, Homo sapiens
tctggagccatacgtgacagaaatggctcagggaactgtt

SEQ ID NO: 1124 - DNA, 40 bp, Homo sapiens
ctgcagtatctgtaaccgaggtctccaggcaccaggagcc

SEQ ID NO: 1125 - DNA, 40 bp, Homo sapiens
ctgcagtatctgtaaccgaggtttctcctctgcctcctac

SEQ ID NO: 1126 - DNA, 40 bp, Homo sapiens
tgatttcaagtttgaacaaggggttggcatctgcacatcc

SEQ ID NO: 1127 - DNA, 40 bp, Homo sapiens
tgatgagactccagacagaggggttggcatctgcacatcc

SEQ ID NO: 1128 - DNA, 40 bp, Homo sapiens
agcgagctcctcagcctcaggcatctgcatctgggaccga

SEQ ID NO: 1129 - DNA, 40 bp, Homo sapiens
ccggggattgccggcgccaggcatctgcatctgggaccga

SEQ ID NO: 1130 - DNA, 40 bp, Homo sapiens
agtttctactagtccagttggtgactctcctattccatct

SEQ ID NO: 1131 - DNA, 40 bp, Homo sapiens
agtttctactagtccagttgggttaccatccattgaccca

SEQ ID NO: 1132 - DNA, 40 bp, Homo sapiens
ggaaaggacagcaagcacaggtgagactgtggagatgaga

SEQ ID NO: 1133 - DNA, 40 bp, Homo sapiens
tgaggtgccctaagcacaaggtgagactgtggagatgaga

SEQ ID NO: 1134 - DNA, 40 bp, Homo sapiens
agttgcatgttgactttagggagtctgtgtgaagcagcac

SEQ ID NO: 1135 - DNA, 40 bp, Homo sapiens
agttgcatgttgactttaggaacgtgaagctcttggagca

SEQ ID NO: 1136 - DNA, 40 bp, Homo sapiens
ccgcccccgttccatccacgggggagctcagtgtgaacac

SEQ ID NO: 1137 - DNA, 40 bp, Homo sapiens
ccgcccccgttccatccacggacgagtgtgaggacgccaa

SEQ ID NO: 1138 - DNA, 40 bp, Homo sapiens
tggagccgaacaacatcgtgctcagcgatgcctgccgctt

SEQ ID NO: 1139 - DNA, 40 bp, Homo sapiens
tggagccgaacaacatcgtggttctgctccagacgagccc

SEQ ID NO: 1140 - DNA, 40 bp, Homo sapiens
gcctggaaagctaccaaaaggagctgtccagacagctggt

SEQ ID NO: 1141 - DNA, 40 bp, Homo sapiens
gcctggaaagctaccaaaagggatctctgcaggagctgtc

SEQ ID NO: 1142 - DNA, 40 bp, Homo sapiens
tgttattgtagattctgggggtggacttctcaaaccaaca

SEQ ID NO: 1143 - DNA, 40 bp, Homo sapiens
tgttattgtagattctgggggctttgatgaactaggtgga

SEQ ID NO: 1144 - DNA, 40 bp, Homo sapiens
ggggaccaagaaaagcagcatggttgcactgaaaagactg

SEQ ID NO: 1145 - DNA, 40 bp, Homo sapiens
ggggaccaagaaaagcagcaccatgaatgacctggtgcag

SEQ ID NO: 1146 - DNA, 40 bp, Homo sapiens
caaaaaagaccaaaactgaggaactccctcggccacagtc

SEQ ID NO: 1147 - DNA, 40 bp, Homo sapiens
caaaaaagaccaaaactgagcaggaactccctcggccaca

SEQ ID NO: 1148 - DNA, 40 bp, Homo sapiens
ccaaagcagagacccaggaggtgtacatggacatcaagat

SEQ ID NO: 1149 - DNA, 40 bp, Homo sapiens
ccaaagcagagacccaggagggagagcccattgctaaaaa

SEQ ID NO: 1150 - DNA, 40 bp, Homo sapiens
gccgaatcacctgatctaaggagattacctggggcaattg

SEQ ID NO: 1151 - DNA, 40 bp, Homo sapiens
acgccgcaagtcctccagaggaacagcagcacaatggacc

SEQ ID NO: 1152 - DNA, 40 bp, Homo sapiens
agcacccatgggtgcagggggaacagcagcacaatggacc

SEQ ID NO: 1153 - DNA, 40 bp, Homo sapiens
aaccagtaacaacggaacctcagagtccagatctgaacga

SEQ ID NO: 1154 - DNA, 40 bp, Homo sapiens
aaccagtaacaacggaacctagtccagatctgaacgatgc

SEQ ID NO: 1155 - DNA, 40 bp, Homo sapiens
gagaccgcgtgcgaggaccgcagcaatgcagagtccctgg

SEQ ID NO: 1156 - DNA, 40 bp, Homo sapiens
gagaccgcgtgcgaggaccgcaatgcagagtccctggaca

SEQ ID NO: 1157 - DNA, 40 bp, Homo sapiens
gtctctggcaagtaatccagaacttcttaatcttccatcc

SEQ ID NO: 1158 - DNA, 40 bp, Homo sapiens
gtctctggcaagtaatccagtaattaagaagaaagttcat

SEQ ID NO: 1159 - DNA, 40 bp, Homo sapiens
aagcatgtagaaagccggaacaggtacttaaaatgaatgc

SEQ ID NO: 1160 - DNA, 40 bp, Homo sapiens
aagcatgtagaaagccggaaggataaagaaatggagaaga

SEQ ID NO: 1161 - DNA, 40 bp, Homo sapiens
agcacccatgggtgcaggggcaagctccagaaaagggact

SEQ ID NO: 1162 - DNA, 40 bp, Homo sapiens
tccacaagagcgaggaggcgaagcgggtgctgcggtatta

SEQ ID NO: 1163 - DNA, 40 bp, Homo sapiens
aggcggtgagtgtcggacagaagcgggtgctgcggtatta

SEQ ID NO: 1164 - DNA, 40 bp, Homo sapiens
tccgccccacagtccacgagactttaccagaatgcaggac

SEQ ID NO: 1165 - DNA, 40 bp, Homo sapiens
ggcggagacatggaccagagactttaccagaatgcaggac

SEQ ID NO: 1166 - DNA, 40 bp, Homo sapiens
ttgatcttcggccccacacgaacagcagagaggggcagca

SEQ ID NO: 1167 - DNA, 40 bp, Homo sapiens
ttgatcttcggccccacacgcagagaggggcagcaggatg

SEQ ID NO: 1168 - DNA, 40 bp, Homo sapiens
gaaaaactttccagccattggggggacaggccccacctcg

SEQ ID NO: 1169 - DNA, 40 bp, Homo sapiens
gaaaaactttccagccattggaggttgtcgggacatttca

SEQ ID NO: 1170 - DNA, 40 bp, Homo sapiens
gcgctcgcccgggcggcagactgtgaggtggagcagtggg

SEQ ID NO: 1171 - DNA, 40 bp, Homo sapiens
ccgcaggatacccgccgaggctgtgaggtggagcagtggg

SEQ ID NO: 1172 - DNA, 40 bp, Homo sapiens
cgggacgacttctacgacaggctcttcgactaccggggcc

SEQ ID NO: 1173 - DNA, 40 bp, Homo sapiens
gcagcatctgccatatacaggctcttcgactaccggggcc

SEQ ID NO: 1174 - DNA, 40 bp, Homo sapiens
actgaagcagcaacacgcctctctgcgtacgtgtcctatg

SEQ ID NO: 1175 - DNA, 40 bp, Homo sapiens
actgaagcagcaacacgcctgctgagattgagagctgctg

SEQ ID NO: 1176 - DNA, 40 bp, Homo sapiens
ctgccggcggagaatataaggagatggacaaaccgtgtgg

SEQ ID NO: 1177 - DNA, 40 bp, Homo sapiens
ctgccggcggagaatataaggtgtgtgtgaccatggaacg

SEQ ID NO: 1178 - DNA, 40 bp, Homo sapiens
caacctctaagactggagcggttcttcttccgcagtggga

SEQ ID NO: 1179 - DNA, 40 bp, Homo sapiens
caacctctaagactggagcgtgggaacatcgagcacccgg

SEQ ID NO: 1180 - DNA, 21 bp, Artificial Sequence
  Description of Artificial Sequence: Synthetic oligonucleotide
gcgagacacactggtattaag

SEQ ID NO: 1181 - DNA, 21 bp, Artificial Sequence
  Description of Artificial Sequence: Synthetic oligonucleotide
tgtggatgagcagcagaaagt

SEQ ID NO: 1182 - DNA, 21 bp, Artificial Sequence
  Description of Artificial Sequence: Synthetic oligonucleotide
gatgagcagcatgaagttcgg

SEQ ID NO: 1183 - DNA, 23 bp, Artificial Sequence
  Description of Artificial Sequence: Synthetic primer
gacttccttctttattgcccttc

SEQ ID NO: 1184 - DNA, 22 bp, Artificial Sequence
  Description of Artificial Sequence: Synthetic primer
agcactgatggtccgaactttc

SEQ ID NO: 1185 - DNA, 21 bp, Artificial Sequence
  Description of Artificial Sequence: Synthetic primer
gtgtgcaaaagcaagaagtcc

SEQ ID NO: 1186 - DNA, 21 bp, Artificial Sequence
  Description of Artificial Sequence: Synthetic primer
gcactgatggtccgaacttca

SEQ ID NO: 1187 - DNA, 25 bp, Artificial Sequence
  Description of Artificial Sequence: Synthetic primer
gcttggcggtgggaaagagaaattg

SEQ ID NO: 1188 - DNA, 27 bp, Artificial Sequence
  Description of Artificial Sequence: Synthetic primer
aaccagtcataccacccaaaggtgttg

SEQ ID NO: 1189 - DNA, 25 bp, Artificial Sequence
  Description of Artificial Sequence: Synthetic primer
ggcacccagcacaatgaagatcaag

SEQ ID NO: 1190 - DNA, 26 bp, Artificial Sequence
  Description of Artificial Sequence: Synthetic primer
actcgtcatactcctgcttgctgatc

SEQ ID NO: 1191 - DNA, 20 bp, Artificial Sequence
  Description of Artificial Sequence: Synthetic primer
actctcttccgcatcgctgt

SEQ ID NO: 1192 - DNA, 20 bp, Artificial Sequence
  Description of Artificial Sequence: Synthetic primer
ccgacgggtttccgatccaa

SEQ ID NO: 1193 - DNA, 18 bp, Artificial Sequence
  Description of Artificial Sequence: Synthetic probe
ctgttgggctcgcggttg

SEQ ID NO: 1194 - DNA, 21 bp, Artificial Sequence
  Description of Artificial Sequence: Synthetic primer
tcttgtctacctctggttcct

SEQ ID NO: 1195 - DNA, 22 bp, Artificial Sequence
  Description of Artificial Sequence: Synthetic primer
ccttcttgttgatgtgcctttc

SEQ ID NO: 1196 - DNA, 24 bp, Artificial Sequence
  Description of Artificial Sequence: Synthetic probe
cagtcttcgcccctcttttcttag

SEQ ID NO: 1197 - DNA, 17 bp, Artificial Sequence
  Description of Artificial Sequence: Synthetic primer
cggtggtgcaagtggaa

SEQ ID NO: 1198 - DNA, 20 bp, Artificial Sequence
  Description of Artificial Sequence: Synthetic primer
gccttggtgtcctcatttct

SEQ ID NO: 1199 - DNA, 24 bp, Artificial Sequence
  Description of Artificial Sequence: Synthetic probe
cttgaggtttcatttccccctccc

SEQ ID NO: 1200 - protein, 1304 aa, Homo sapiens
MAKIAKTHEDIEAQIREIQGKKAALDEAQGVGLDSTGYYDQEIYGGSDSRFAGYVTSIAATELEDDDDDYSSSTSLLGQKKPGYHAPVALLNDIPQSTEQYDPFAEHRPPKIADREDEYKKHRRTMIISPERLDPFADGGKTPDPKMNARTYMDVMREQHLTKEEREIRQQLAEKAKAGELKVVNGAAASQPPSKRKRRWDQTADQTPGATPKKLSSWDQAETPGHTPSLRWDETPGRAKGSETPGATPGSKIWDPTPSHTPAGAATPGRGDTPGHATPGHGGATSSARKNRWDETPKTERDTPGHGSGWAETPRTDRGGDSIGETPTPGASKRKSRWDETPASQMGGSTPVLTPGKTPIGTPAMNMATPTPGHIMSMTPEQLQAWRWEREIDERNRPLSDEELDAMFPEGYKVLPPPAGYVPIRTPARKLTATPTPLGGMTGFHMQTEDRTMKSVNDQPSGNLPFLKPDDIQYFDKLLVDVDESTLSPEEQKERKIMKLLLKIKNGTPPMRKAALRQITDKAREFGAGPLFNQILPLLMSPTLEDQERHLLVKVIDRILYKLDDLVRPYVHKILVVIEPLLIDEDYYARVEGREIISNLAKAAGLATMISTMRPDIDNMDEYVRNTTARAFAVVASALGIPSLLPFLKAVCKSKKSWQARHTGIKIVQQIAILMGCAILPHLRSLVEIIEHGLVDEQQKVRTISALAIAALAEAATPYGIESFDSVLKPLWKGIRQHRGKGLAAFLKAIGYLIPLMDAEYANYYTREVMLILIREFQSPDEEMKKIVLKVVKQCCGTDGVEANYIKTEILPPFFKHFWQHRMALDRRNYRQLVDTTVELANKVGAAEIISRIVDDLKDEAEQYRKMVMETIEKIMGNLGAADIDHKLEEQLIDGILYAFQEQTTEDSVMLNGFGTVVNALGKRVKPYLPQICGTVLWRLNNKSAKVRQQAADLISRTAVVMKTCQEEKLMGHLGVVLYEYLGEEYPEVLGSILGALKAIVNVIGMHKMTPPIKDLLPRLTPILKNRHEKVQENCIDLVGRIADRGAEYVSAREWMRICFELLELLKAHKKAIRRATVNTFGYIAKAIGPHDVLATLLNNLKVQERQNRVCTTVAIAIVAETCSPFTVLPALMNEYRVPELNVQNGVLKSLSFLFEYIGEMGKDYIYAVTPLLEDALMDRDLVHRQTASAVVQHMSLGVYGFGCEDSLNHLLNYVWPNVFETSPHVIQAVMGALEGLRVAIGPCRMLQYCLQGLFHPARKVRDVYWKIYNSIYIGSQDALIAHYPRIYNDDKNTYIRYELDYIL